European Patent Application EP 4 715 057 A1, published March 25, 2026. Title: 腺相关病毒衣壳蛋白、包含其的腺相关病毒及应用. Applicant: 杭州新昶基因技术有限公司. The sequence listing filed with the application follows.

SEQUENCE LISTING (27 sequences)

SEQ ID NO: 1 - DNA, 7327 bp, synthetic construct
  source 1..7327: mol_type = other DNA
gacaggtttcccgactggaaagcgggcagtgagcgcaacgcaattaatgtgagttagctcactcattaggcaccccaggctttacactttatgcttccggctcgtatgttgtgtggaattgtgagcggataacaatttcacacaggaaacagctatgaccatgattacgccaagcgcgccgatatcgttaacgccccgcgccggccgctctagaactagtggatcccccggaagatcagaagttcctattccgaagttcctattctctagaaagtataggaacttctgatctgcgcagccgccatgccggggttttacgagattgtgattaaggtccccagcgaccttgacgagcatctgcccggcatttctgacagctttgtgaactgggtggccgagaaggaatgggagttgccgccagattctgacatggatctgaatctgattgagcaggcacccctgaccgtggccgagaagctgcagcgcgactttctgacggaatggcgccgtgtgagtaaggccccggaggcccttttctttgtgcaatttgagaagggagagagctacttccacatgcacgtgctcgtggaaaccaccggggtgaaatccatggttttgggacgtttcctgagtcagattcgcgaaaaactgattcagagaatttaccgcgggatcgagccgactttgccaaactggttcgcggtcacaaagaccagaaatggcgccggaggcgggaacaaggtggtggatgagtgctacatccccaattacttgctccccaaaacccagcctgagctccagtgggcgtggactaatatggaacagtatttaagcgcctgtttgaatctcacggagcgtaaacggttggtggcgcagcatctgacgcacgtgtcgcagacgcaggagcagaacaaagagaatcagaatcccaattctgatgcgccggtgatcagatcaaaaacttcagccaggtacatggagctggtcgggtggctcgtggacaaggggattacctcggagaagcagtggatccaggaggaccaggcctcatacatctccttcaatgcggcctccaactcgcggtcccaaatcaaggctgccttggacaatgcgggaaagattatgagcctgactaaaaccgcccccgactacctggtgggccagcagcccgtggaggacatttccagcaatcggatttataaaattttggaactaaacgggtacgatccccaatatgcggcttccgtctttctgggatgggccacgaaaaagttcggcaagaggaacaccatctggctgtttgggcctgcaactaccgggaagaccaacatcgcggaggccatagcccacactgtgcccttctacgggtgcgtaaactggaccaatgagaactttcccttcaacgactgtgtcgacaagatggtgatctggtgggaggaggggaagatgaccgccaaggtcgtggagtcggccaaagccattctcggaggaagcaaggtgcgcgtggaccagaaatgcaagtcctcggcccagatagacccgactcccgtgatcgtcacctccaacaccaacatgtgcgccgtgattgacgggaactcaacgaccttcgaacaccagcagccgttgcaagaccggatgttcaaatttgaactcacccgccgtctggatcatgactttgggaaggtcaccaagcaggaagtcaaagactttttccggtgggcaaaggatcacgtggttgaggtggagcatgaattctacgtcaaaaagggtggagccaagaaaagacccgcccccagtgacgcagatataagtgagcccaaacgggtgcgcgagtcagttgcgcagccatcgacgtcagacgcggaagcttcgatcaactacgcagacaggtaccaaaacaaatgttctcgtcacgtgggcatgaatctgatgctgtttccctgcagacaatgcgagagaatgaatcagaattcaaatatctgcttcactcacggacagaaagactgtttagagtgctttcccgtgtcagaatctcaacccgtttctgtcgtcaaaaaggcgtatcagaaactgtgctacattcatcatatcatgggaaaggtgccagacgcttgcactgcctgcgatctggtcaatgtggatttggatgactgcatctttgaacaataaatgatttaaatcaggtatggctgccgatggttatcttccagattggctcgaggacactctctctgaaggaataagacagtggtggaagctcaaacctggcccaccaccaccaaagcccgcagagcggcataaggacgacagcaggggtcttgtgcttcctgggtacaagtacctcggacccttcaacggactcgacaagggagagccggtcaacgaggcagacgccgcggccctcgagcacgacaaagcctacgaccggcagctcgacagcggagacaacccgtacctcaagtacaaccacgccgacgcggagtttcaggagcgccttaaagaagatacgtcttttgggggcaacctcggacgagcagtcttccaggcgaaaaagagggttcttgaacctctgggcctggttgaggaacctgttaagacggctccgggaaaaaagaggccggtagagcactctcctgtggagccagactcctcctcgggaaccggaaaggcgggccagcagcctgcaagaaaaagattgaattttggtcagactggagacgcagactcagtacctgacccccagcctctcggacagccaccagcagccccctctggtctgggaactaatacgatggctacaggcagtggcgcaccaatggcagacaataacgagggcgccgacggagtgggtaattcctcgggaaattggcattgcgattccacatggatgggcgacagagtcatcaccaccagcacccgaacctgggccctgcccacctacaacaaccacctctacaaacaaatttccagccaatcaggagcctcgaacgacaatcactactttggctacagcaccccttgggggtattttgacttcaacagattccactgccacttttcaccacgtgactggcaaagactcatcaacaacaactggggattccgacccaagagactcaacttcaagctctttaacattcaagtcaaagaggtcacgcagaatgacggtacgacgacgattgccaataaccttaccagcacggttcaggtgtttactgactcggagtaccagctcccgtacgtcctcggctcggcgcatcaaggatgcctcccgccgttcccagcagacgtcttcatggtgccacagtatggatacctcaccctgaacaacgggagtcaggcagtaggacgctcttcattttactgcctggagtactttccttctcagatgctgcgtaccggaaacaactttaccttcagctacacttttgaggacgttcctttccacagcagctacgctcacagccagagtctggaccgtctcatgaatcctctcatcgaccagtacctgtattacttgagcagaacaaacactccaagtggaaccaccacgcagtcaaggcttcagttttctcaggccggagcgagtgacattcgggaccagtctaggaactggcttcctggaccctgttaccgccagcagcgagtatcaaagacatctgcggataacaacaacagtgaatactcgtggactggagctaccaagtaccacctcaatggcagagactctctggtgaatccgggcccggccatggcaagccacaaggacgatgaagaaaagttttttcctcagagcggggttctcatctttgggaagcaaggctcagagaaaacaaatgtggacattgaaaaggtcatgattacagacgaagaggaaatcaggacaaccaatcccgtggctacggagcagtatggttctgtatctaccaacctccagagaggcaacagacaagcagctaccgcagatgtcaacacacaaggcgttcttccaggcatggtctggcaggacagagatgtgtaccttcaggggcccatctgggcaaagattccacacacggacggacattttcacccctctcccctcatgggtggattcggacttaaacaccctcctccacagattctcatcaagaacaccccggtacctgcgaatccttcgaccaccttcagtgcggcaaagtttgcttccttcatcacacagtactccacgggacaggtcagcgtggagatcgagtgggagctgcagaaggaaaacagcaaacgctggaatcccgaaattcagtacacttccaactacaacaagtctgttaatgtggactttactgtggacactaatggcgtgtattcagagcctcgccccattggcaccagatacctgactcgtaatctgtaattgcttgttaatcaataaaccgtttaattcgtttcagttgaactttggtctctgcgtatttctttcttatctagtttccatggctacgtagataagtagcatggcgggttaatcattaactacagcccgggcgtttaaacagcgggcggaggggtggagtcgtgacgtgaattacgtcatagggttagggaggtcctgtattagaggtcacgtgagtgttttgcgacattttgcgacaccatgtggtctcgctgggggggggggcccgagtgagcacgcagggtctccattttgaagcgggaggtttgaacgagcgctggcgcgctcactggccgtcgttttacaacgtcgtgactgggaaaaccctggcgttacccaacttaatcgccttgcagcacatccccctttcgccagctggcgtaatagcgaagaggcccgcaccgatcgcccttcccaacagttgcgcagcctgaatggcgaatggaaattgtaagcgttaatattttgttaaaattcgcgttaaatttttgttaaatcagctcatttttttaaccaataggccgaaatcggcaaaatcccttataaatcaaaagaatagaccgagatagggttgagtgttgttccagtttggaacaagagtccactattaagaacgtggactccaacgtcaaagggcgaaaaaccgtctatcagggcgatggcccactacgtgaaccatcaccctaatcaagttttttggggtcgaggtgccgtaaagcactaaatcggaaccctaaagggagcccccgatttagagcttgacggggaaagccggcgaacgtggcgagaaaggaagggaagaaagcgaaaggagcgggcgctagggcgctggcaagtgtagcggtcacgctgcgcgtaaccaccacacccgccgcgcttaatgcgccgctacagggcgcgtcaggtggcacttttcggggaaatgtgcgcggaacccctatttgtttatttttctaaatacattcaaatatgtatccgctcatgagacaataaccctgataaatgcttcaataatattgaaaaaggaagagtatgagtattcaacatttccgtgtcgcccttattcccttttttgcggcattttgccttcctgtttttgctcacccagaaacgctggtgaaagtaaaagatgctgaagatcagttgggtgcacgagtgggttacatcgaactggatctcaacagcggtaagatccttgagagttttcgccccgaagaacgttttccaatgatgagcacttttaaagttctgctatgtggcgcggtattatcccgtattgacgccgggcaagagcaactcggtcgccgcatacactattctcagaatgacttggttgagtactcaccagtcacagaaaagcatcttacggatggcatgacagtaagagaattatgcagtgctgccataaccatgagtgataacactgcggccaacttacttctgacaacgatcggaggaccgaaggagctaaccgcttttttgcacaacatgggggatcatgtaactcgccttgatcgttgggaaccggagctgaatgaagccataccaaacgacgagcgtgacaccacgatgcctgtagcaatggcaacaacgttgcgcaaactattaactggcgaactacttactctagcttcccggcaacaattaatagactggatggaggcggataaagttgcaggaccacttctgcgctcggcccttccggctggctggtttattgctgataaatctggagccggtgagcgtgggtctcgcggtatcattgcagcactggggccagatggtaagccctcccgtatcgtagttatctacacgacggggagtcaggcaactatggatgaacgaaatagacagatcgctgagataggtgcctcactgattaagcattggtaactgtcagaccaagtttactcatatatactttagattgatttaaaacttcatttttaatttaaaaggatctaggtgaagatcctttttgataatctcatgaccaaaatcccttaacgtgagttttcgttccactgagcgtcagaccccgtagaaaagatcaaaggatcttcttgagatcctttttttctgcgcgtaatctgctgcttgcaaacaaaaaaaccaccgctaccagcggtggtttgtttgccggatcaagagctaccaactctttttccgaaggtaactggcttcagcagagcgcagataccaaatactgttcttctagtgtagccgtagttaggccaccacttcaagaactctgtagcaccgcctacatacctcgctctgctaatcctgttaccagtggctgctgccagtggcgataagtcgtgtcttaccgggttggactcaagacgatagttaccggataaggcgcagcggtcgggctgaacggggggttcgtgcacacagcccagcttggagcgaacgacctacaccgaactgagatacctacagcgtgagctatgagaaagcgccacgcttcccgaagggagaaaggcggacaggtatccggtaagcggcagggtcggaacaggagagcgcacgagggagcttccagggggaaacgcctggtatctttatagtcctgtcgggtttcgccacctctgacttgagcgtcgatttttgtgatgctcgtcaggggggcggagcctatggaaaaacgccagcaacgcggcctttttacggttcctggccttttgctggccttttgctcacatgttctttcctgcgttatcccctgattctgtggataaccgtattaccgcctttgagtgagctgataccgctcgccgcagccgaacgaccgagcgcagcgagtcagtgagcgaggaagcggaagagcgcccaatacgcaaaccgcctctccccgcgcgttggccgattcattaatgcagctggcac

SEQ ID NO: 2 - DNA, 7468 bp, synthetic construct
  source 1..7468: mol_type = other DNA
agggttgagtgttgttccagtttggaacaagagtccactattaaagaacgtggactccaacgtcaaagggcgaaaaaccgtctatcagggcgatggcccactacgtgaaccatcaccctaatcaagttttttggggtcgaggtgccgtaaagcactaaatcggaaccctaaagggagcccccgatttagagcttgacggggaaagccggcgaacgtggcgagaaaggaagggaagaaagcgaaaggagcgggcgctagggcgctggcaagtgtagcggtcacgctgcgcgtaaccaccacacccgccgcgcttaatgcgccgctacagggcgcgtccattcgccattcaggctgcgcaactgttgggaagggcgatcggtgcgggcctcttcgctattacgccagctggcgaaagggggatgtgctgcaaggcgattaagttgggtaacgccagggttttcccagtcacgacgttgtaaaacgacggccagtgaattgtaatacgactcactatagggcgaattcgagctcggtacccctagaggtcctgtattagaggtcacgtgagtgttttgcgacattttgcgacaccatgtggtcacgctgggtatttaagcccgagtgagcacgcagggtctccattttgaagcgggaggtttgaacgcgcagccaccacgccggggttttacgagattgtgattaaggtccccagcgaccttgacgagcatctgcccggcatttctgacagctttgtgaactgggtggccgagaaggaatgggagttgccgccagattctgacatggatctgaatctgattgagcaggcacccctgaccgtggccgagaagctgcagcgcgactttctgacggaatggcgccgtgtgagtaaggccccggaggcccttttctttgtgcaatttgagaagggagagagctacttccacatgcacgtgctcgtggaaaccaccggggtgaaatccatggttttgggacgtttcctgagtcagattcgcgaaaaactgattcagagaatttaccgcgggatcgagccgactttgccaaactggttcgcggtcacaaagaccagaaatggcgccggaggcgggaacaaggtggtggatgagtgctacatccccaattacttgctccccaaaacccagcctgagctccagtgggcgtggactaatatggaacagtatttaagcgcctgtttgaatctcacggagcgtaaacggttggtggcgcagcatctgacgcacgtgtcgcagacgcaggagcagaacaaagagaatcagaatcccaattctgatgcgccggtgatcagatcaaaaacttcagccaggtacatggagctggtcgggtggctcgtggacaaggggattacctcggagaagcagtggatccaggaggaccaggcctcatacatctccttcaatgcggcctccaactcgcggtcccaaatcaaggctgccttggacaatgcgggaaagattatgagcctgactaaaaccgcccccgactacctggtgggccagcagcccgtggaggacatttccagcaatcggatttataaaattttggaactaaacgggtacgatccccaatatgcggcttccgtctttctgggatgggccacgaaaaagttcggcaagaggaacaccatctggctgtttgggcctgcaactaccgggaagaccaacatcgcggaggccatagcccacactgtgcccttctacgggtgcgtaaactggaccaatgagaactttcccttcaacgactgtgtcgacaagatggtgatctggtgggaggagggcaagatgacggccaaggtcgtggagtccgccaaggccattctcggcggcagcaaggtgcgcgtggaccaaaagtgcaagtcgtccgcccagatcgatcccacccccgtgatcgtcacctccaacaccaacatgtgcgccgtgattgacgggaacagcaccaccttcgagcaccagcagccgttgcaggaccggatgttcaaatttgaactcacccgccgtctggagcatgactttggcaaggtgacaaagcaggaagtcaaagagttcttccgctgggcgcaggatcacgtgaccgaggtggcgcatgagttctacgtcagaaagggtggagccaacaagagacccgcccccgatgacgcggataaaagcgagcccaagcgggcctgcccctcagtcgcggatccatcgacgtcagacgcggaaggagctccggtggactttgccgacaggtaccaaaacaaatgttctcgtcacgcgggcatgcttcagatgctgtttccctgcaaaacatgcgagagaatgaatcagaatttcaacatttgcttcacgcacgggaccagagactgttcagaatgtttccccggcgtgtcagaatctcaaccggtcgtcagaaagaggacgtatcggaaactctgtgccattcatcatctgctggggcgggctcccgagattgcttgctcggcctgcgatctggtcaacgtggatctggatgactgtgtttctgagcaataaatgacttaaaccaggtatggctgccgatggttatcttccagattggctcgaggacaacctctctgagggcattcgcgagtggtgggacttgaaacctggagccccgaaacccaaagccaaccagcaaaagcaggacgacggccggggtctggtgcttcctggctacaagtacctcggacccttcaacggactcgacaagggggagcccgtcaacgcggcggatgcagcggccctcgagcacgacaaggcctacgaccagcagctcaaagcgggtgacaatccgtacctgcggtataaccacgccgacgccgagtttcaggagcgtctgcaagaagatacgtcttttgggggcaacctcgggcgagcagtcttccaggccaagaagagggttctcgaaccttttggtctggttgaggaaggtgctaagacggctcctggaaagaaacgtccggtagagcagtcgccacaagagccagactcctcctcgggcattggcaagacaggccagcagcccgctaaaaagagactcaattttggtcagactggcgactcagagtcagtccccgacccacaacctctcggagaacctccagcaacccccgctgctgtgggacctactacaatggcttcaggcggtggcgcaccaatggcagacaataacgaaggcgccgacggagtgggtaatgcctcaggaaattggcattgcgattccacatggctgggcgacagagtcatcaccaccagcacccgaacatgggccttgcccacctataacaaccacctctacaagcaaatctccagtgcttcaacgggggccagcaacgacaaccactacttcggctacagcaccccctgggggtattttgatttcaacagattccactgccatttctcaccacgtgactggcagcgactcatcaacaacaattggggattccggcccaagagactcaacttcaagctcttcaacatccaagtcaaggaggtcacgacgaatgatggcgtcacgaccatcgctaataaccttaccagcacggttcaagtcttctcggactcggagtaccagttgccgtacgtcctcggctctgcgcaccagggctgcctccctccgttcccggcggacgtgttcatgattccgcagtacggctacctaacgctcaacaatggcagccaggcagtgggacggtcatccttttactgcctggaatatttcccatcgcagatgctgagaacgggcaataactttaccttcagctacaccttcgaggacgtgcctttccacagcagctacgcgcacagccagagcctggaccggctgatgaatcctctcatcgaccagtacctgtattacctgaacagaactcagaatcagtccggaagtgcccaaaacaaggacttgctgtttagccgggggtctccagctggcatgtctgttcagcccaaaaactggctacctggaccctgttaccggcagcagcgcgtttctaaaacaaaaacagacaacaacaacagcaactttacctggactggtgcttcaaaatataaccttaatgggcgtgaatctataatcaaccctggcactgctatggcctcacacaaagacgacaaagacaagttctttcccatgagcggtgtcatgatttttggaaaggagagcgccggagcttcaaacactgcattggacaatgtcatgatcacagacgaagaggaaatcaaagccactaaccccgtggccaccgaaagatttgggactgtggcagtcaatctccagagcagcagcacagaccctgcgaccggagatgtgcatgttatgggagccttacctggaatggtgtggcaagacagagacgtatacctgcagggtcctatttgggccaaaattcctcacacggatggacactttcacccgtctcctctcatgggcggctttggacttaagcacccgcctcctcagatcctcatcaaaaacacgcctgttcctgcgaatcctccggcagagttttcggctacaaagtttgcttcattcatcacccagtattccacaggacaagtgagcgtggagattgaatgggagctgcagaaagaaaacagcaaacgctggaatcccgaagtgcagtatacatctaactatgcaaaatctgccaacgttgatttcactgtggacaacaatggactttatactgagcctcgccccattggcacccgttacctcacccgtcccctgtaattgtctgttaatcaataaaccggttgattcgtttcagttgaactttggtctcgcggccgctcgataagcttttgttccctttagtgagggttaatttcgagcttggcgtaatcatggtcatagctgtttcctgtgtgaaattgttatccgctcacaattccacacaacatacgagccggaagcataaagtgtaaagcctggggtgcctaatgagtgagctaactcacattaattgcgttgcgctcactgcccgctttccagtcgggaaacctgtcgtgccagctgcattaatgaatcggccaacgcgcggggagaggcggtttgcgtattgggcgctcttccgcttcctcgctcactgactcgctgcgctcggtcgttcggctgcggcgagcggtatcagctcactcaaaggcggtaatacggttatccacagaatcaggggataacgcaggaaagaacatgtgagcaaaaggccagcaaaaggccaggaaccgtaaaaaggccgcgttgctggcgtttttccataggctccgcccccctgacgagcatcacaaaaatcgacgctcaagtcagaggtggcgaaacccgacaggactataaagataccaggcgtttccccctggaagctccctcgtgcgctctcctgttccgaccctgccgcttaccggatacctgtccgcctttctcccttcgggaagcgtggcgctttctcatagctcacgctgtaggtatctcagttcggtgtaggtcgttcgctccaagctgggctgtgtgcacgaaccccccgttcagcccgaccgctgcgccttatccggtaactatcgtcttgagtccaacccggtaagacacgacttatcgccactggcagcagccactggtaacaggattagcagagcgaggtatgtaggcggtgctacagagttcttgaagtggtggcctaactacggctacactagaagaacagtatttggtatctgcgctctgctgaagccagttaccttcggaaaaagagttggtagctcttgatccggcaaacaaaccaccgctggtagcggtggtttttttgtttgcaagcagcagattacgcgcagaaaaaaaggatctcaagaagatcctttgatcttttctacggggtctgacgctcagtggaacgaaaactcacgttaagggattttggtcatgagattatcaaaaaggatcttcacctagatccttttaaattaaaaatgaagttttaaatcaatctaaagtatatatgagtaaacttggtctgacagttaccaatgcttaatcagtgaggcacctatctcagcgatctgtctatttcgttcatccatagttgcctgactccccgtcgtgtagataactacgatacgggagggcttaccatctggccccagtgctgcaatgataccgcgagacccacgctcaccggctccagatttatcagcaataaaccagccagccggaagggccgagcgcagaagtggtcctgcaactttatccgcctccatccagtctattaattgttgccgggaagctagagtaagtagttcgccagttaatagtttgcgcaacgttgttgccattgctacaggcatcgtggtgtcacgctcgtcgtttggtatggcttcattcagctccggttcccaacgatcaaggcgagttacatgatcccccatgttgtgcaaaaaagcggttagctccttcggtcctccgatcgttgtcagaagtaagttggccgcagtgttatcactcatggttatggcagcactgcataattctcttactgtcatgccatccgtaagatgcttttctgtgactggtgagtactcaaccaagtcattctgagaatagtgtatgcggcgaccgagttgctcttgcccggcgtcaatacgggataataccgcgccacatagcagaactttaaaagtgctcatcattggaaaacgttcttcggggcgaaaactctcaaggatcttaccgctgttgagatccagttcgatgtaacccactcgtgcacccaactgatcttcagcatcttttactttcaccagcgtttctgggtgagcaaaaacaggaaggcaaaatgccgcaaaaaagggaataagggcgacacggaaatgttgaatactcatactcttcctttttcaatattattgaagcatttatcagggttattgtctcatgagcggatacatatttgaatgtatttagaaaaataaacaaataggggttccgcgcacatttccccgaaaagtgccacctgacgtctaagaaaccattattatcatgacattaacctataaaaataggcgtatcacgaggccctttcgtctcgcgcgtttcggtgatgacggtgaaaacctctgacacatgcagctcccggagacggtcacagcttgtctgtaagcggatgccgggagcagacaagcccgtcagggcgcgtcagcgggtgttggcgggtgtcggggctggcttaactatgcggcatcagagcagattgtactgagagtgcaccatatgcggtgtgaaataccgcacagatgcgtaaggagaaaataccgcatcaggaaattgtaagcgttaatattttgttaaaattcgcgttaaatttttgttaaatcagctcattttttaaccaataggccgaaatcggcaaaatcccttataaatcaaaagaatagaccgagat

SEQ ID NO: 3 - DNA, 7330 bp, synthetic construct
  source 1..7330: mol_type = other DNA
ctgttgggaagggcgatcggtgcgggcctcttcgctattacgccagctggcgaaagggggatgtgctgcaaggcgattaagttgggtaacgccagggttttcccagtcacgacgttgtaaaacgacggccagtgagcgcgcgtaatacgactcactatagggcgaattgggtaccgggccccccctcgatcgaggtcgacggtatcgggggagctcgcagggtctccattttgaagcgggaggtttgaacgcgcagccgccatgccggggttttacgagattgtgattaaggtccccagcgaccttgacgagcatctgcccggcatttctgacagctttgtgaactgggtggccgagaaggaatgggagttgccgccagattctgacatggatctgaatctgattgagcaggcacccctgaccgtggccgagaagctgcagcgcgactttctgacggaatggcgccgtgtgagtaaggccccggaggctcttttctttgtgcaatttgagaagggagagagctacttccacatgcacgtgctcgtggaaaccaccggggtgaaatccatggttttgggacgtttcctgagtcagattcgcgaaaaactgattcagagaatttaccgcgggatcgagccgactttgccaaactggttcgcggtcacaaagaccagaaatggcgccggaggcgggaacaaggtggtggatgagtgctacatccccaattacttgctccccaaaacccagcctgagctccagtgggcgtggactaatatggaacagtatttaagcgcctgtttgaatctcacggagcgtaaacggttggtggcgcagcatctgacgcacgtgtcgcagacgcaggagcagaacaaagagaatcagaatcccaattctgatgcgccggtgatcagatcaaaaacttcagccaggtacatggagctggtcgggtggctcgtggacaaggggattacctcggagaagcagtggatccaggaggaccaggcctcatacatctccttcaatgcggcctccaactcgcggtcccaaatcaaggctgccttggacaatgcgggaaagattatgagcctgactaaaaccgcccccgactacctggtgggccagcagcccgtggaggacatttccagcaatcggatttataaaattttggaactaaacgggtacgatccccaatatgcggcttccgtctttctgggatgggccacgaaaaagttcggcaagaggaacaccatctggctgtttgggcctgcaactaccgggaagaccaacatcgcggaggccatagcccacactgtgcccttctacgggtgcgtaaactggaccaatgagaactttcccttcaacgactgtgtcgacaagatggtgatctggtgggaggaggggaagatgaccgccaaggtcgtggagtcggccaaagccattctcggaggaagcaaggtgcgcgtggaccagaaatgcaagtcctcggcccagatagacccgactcccgtgatcgtcacctccaacaccaacatgtgcgccgtgattgacgggaactcaacgaccttcgaacaccagcagccgttgcaagaccggatgttcaaatttgaactcacccgccgtctggatcatgactttgggaaggtcaccaagcaggaagtcaaagactttttccggtgggcaaaggatcacgtggttgaggtggagcatgaattctacgtcaaaaagggtggagccaagaaaagacccgcccccagtgacgcagatataagtgagcccaaacgggtgcgcgagtcagttgcgcagccatcgacgtcagacgcggaagcttcgatcaactacgcggacaggtaccaaaacaaatgttctcgtcacgtgggcatgaatctgatgctgtttccctgcagacaatgcgagagactgaatcagaattcaaatatctgcttcactcacggtgtcaaagactgtttagagtgctttcccgtgtcagaatctcaacccgtttctgtcgtcaaaaaggcgtatcagaaactgtgctacattcatcacatcatgggaaaggtgccagacgcttgcactgcttgcgacctggtcaatgtggacttggatgactgtgtttctgaacaataaatgacttaaaccaggtatggctgccgatggttatcttccagattggctcgaggacaaccttagtgaaggaattcgcgagtggtgggctttgaaacctggagcccctcaacccaaggcaaatcaacaacatcaagacaacgctcgaggtcttgtgcttccgggttacaaataccttggacccggcaacggactcgacaagggggagccggtcaacgcagcagacgcggcggccctcgagcacgacaaggcctacgaccagcagctcaaggccggagacaacccgtacctcaagtacaaccacgccgacgccgagttccaggagcggctcaaagaagatacgtcttttgggggcaacctcgggcgagcagtcttccaggccaaaaagaggcttcttgaacctcttggtctggttgaggaagcggctaagacggctcctggaaagaagaggcctgtagagcagtctcctcaggaaccggactcctccgcgggtattggcaaatcgggtgcacagcccgctaaaaagagactcaatttcggtcagactggcgacacagagtcagtcccagaccctcaaccaatcggagaacctcccgcagccccctcaggtgtgggatctcttacaatggcttcaggtggtggcgcaccagtggcagacaataacgaaggtgccgatggagtgggtagttcctcgggaaattggcattgcgattcccaatggctgggggacagagtcatcaccaccagcacccgaacctgggccctgcccacctacaacaatcacctctacaagcaaatctccaacagcacatctggaggatcttcaaatgacaacgcctacttcggctacagcaccccctgggggtattttgacttcaacagattccactgccacttctcaccacgtgactggcagcgactcatcaacaacaactggggattccggcctaagcgactcaacttcaagctcttcaacattcaggtcaaagaggttacggacaacaatggagtcaagaccatcgccaataaccttaccagcacggtccaggtcttcacggactcagactatcagctcccgtacgtgctcgggtcggctcacgagggctgcctcccgccgttcccagcggacgttttcatgattcctcagtacgggtatctgacgcttaatgatggaagccaggccgtgggtcgttcgtccttttactgcctggaatatttcccgtcgcaaatgctaagaacgggtaacaacttccagttcagctacgagtttgagaacgtacctttccatagcagctacgctcacagccaaagcctggaccgactaatgaatccactcatcgaccaatacttgtactatctctcaaagactattaacggttctggacagaatcaacaaacgctaaaattcagtgtggccggacccagcaacatggctgtccagggaagaaactacatacctggacccagctaccgacaacaacgtgtctcaaccactgtgactcaaaacaacaacagcgaatttgcttggcctggagcttcttcttgggctctcaatggacgtaatagcttgatgaatcctggacctgctatggccagccacaaagaaggagaggaccgtttctttcctttgtctggatctttaatttttggcaaacaaggaactggaagagacaacgtggatgcggacaaagtcatgataaccaacgaagaagaaattaaaactactaacccggtagcaacggagtcctatggacaagtggccacaaaccaccagagtgcccaagcacaggcgcagaccggctgggttcaaaaccaaggaatacttccgggtatggtttggcaggacagagatgtgtacctgcaaggacccatttgggccaaaattcctcacacggacggcaactttcacccttctccgctgatgggagggtttggaatgaagcacccgcctcctcagatcctcatcaaaaacacacctgtacctgcggatcctccaacggccttcaacaaggacaagctgaactctttcatcacccagtattctactggccaagtcagcgtggagatcgagtgggagctgcagaaggaaaacagcaagcgctggaacccggagatccagtacacttccaactattacaagtctaataatgttgaatttgctgttaatactgaaggtgtatatagtgaaccccgccccattggcaccagatacctgactcgtaatctgtaattgcttgttaatcaataaaccgtttaattcgtttcagttgaactttggtctctgcgaagggcgaattcgtttaaacctgcaggactagaggtcctgtattagaggtcacgtgagtgttttgcgacattttgcgacaccatgtggtcacgctgggtatttaagcccgagtgagcacgcagggtctccattttgaagcgggaggtttgaacgcgcagccgccaagccgaattctgcagatatccatcacactggcggccgctcgactagagcggccgccaccgcggtggagctccagcttttgttccctttagtgagggttaattgcgcgcttggcgtaatcatggtcatagctgtttcctgtgtgaaattgttatccgctcacaattccacacaacatacgagccggaagcataaagtgtaaagcctggggtgcctaatgagtgagctaactcacattaattgcgttgcgctcactgcccgctttccagtcgggaaacctgtcgtgccagctgcattaatgaatcggccaacgcgcggggagaggcggtttgcgtattgggcgctcttccgcttcctcgctcactgactcgctgcgctcggtcgttcggctgcggcgagcggtatcagctcactcaaaggcggtaatacggttatccacagaatcaggggataacgcaggaaagaacatgtgagcaaaaggccagcaaaaggccaggaaccgtaaaaaggccgcgttgctggcgtttttccataggctccgcccccctgacgagcatcacaaaaatcgacgctcaagtcagaggtggcgaaacccgacaggactataaagataccaggcgtttccccctggaagctccctcgtgcgctctcctgttccgaccctgccgcttaccggatacctgtccgcctttctcccttcgggaagcgtggcgctttctcatagctcacgctgtaggtatctcagttcggtgtaggtcgttcgctccaagctgggctgtgtgcacgaaccccccgttcagcccgaccgctgcgccttatccggtaactatcgtcttgagtccaacccggtaagacacgacttatcgccactggcagcagccactggtaacaggattagcagagcgaggtatgtaggcggtgctacagagttcttgaagtggtggcctaactacggctacactagaagaacagtatttggtatctgcgctctgctgaagccagttaccttcggaaaaagagttggtagctcttgatccggcaaacaaaccaccgctggtagcggtggtttttttgtttgcaagcagcagattacgcgcagaaaaaaaggatctcaagaagatcctttgatcttttctacggggtctgacgctcagtggaacgaaaactcacgttaagggattttggtcatgagattatcaaaaaggatcttcacctagatccttttaaattaaaaatgaagttttaaatcaatctaaagtatatatgagtaaacttggtctgacagttaccaatgcttaatcagtgaggcacctatctcagcgatctgtctatttcgttcatccatagttgcctgactccccgtcgtgtagataactacgatacgggagggcttaccatctggccccagtgctgcaatgataccgcgagacccacgctcaccggctccagatttatcagcaataaaccagccagccggaagggccgagcgcagaagtggtcctgcaactttatccgcctccatccagtctattaattgttgccgggaagctagagtaagtagttcgccagttaatagtttgcgcaacgttgttgccattgctacaggcatcgtggtgtcacgctcgtcgtttggtatggcttcattcagctccggttcccaacgatcaaggcgagttacatgatcccccatgttgtgcaaaaaagcggttagctccttcggtcctccgatcgttgtcagaagtaagttggccgcagtgttatcactcatggttatggcagcactgcataattctcttactgtcatgccatccgtaagatgcttttctgtgactggtgagtactcaaccaagtcattctgagaatagtgtatgcggcgaccgagttgctcttgcccggcgtcaatacgggataataccgcgccacatagcagaactttaaaagtgctcatcattggaaaacgttcttcggggcgaaaactctcaaggatcttaccgctgttgagatccagttcgatgtaacccactcgtgcacccaactgatcttcagcatcttttactttcaccagcgtttctgggtgagcaaaaacaggaaggcaaaatgccgcaaaaaagggaataagggcgacacggaaatgttgaatactcatactcttcctttttcaatattattgaagcatttatcagggttattgtctcatgagcggatacatatttgaatgtatttagaaaaataaacaaataggggttccgcgcacatttccccgaaaagtgccacctaaattgtaagcgttaatattttgttaaaattcgcgttaaatttttgttaaatcagctcattttttaaccaataggccgaaatcggcaaaatcccttataaatcaaaagaatagaccgagatagggttgagtgttgttccagtttggaacaagagtccactattaaagaacgtggactccaacgtcaaagggcgaaaaaccgtctatcagggcgatggcccactacgtgaaccatcaccctaatcaagttttttggggtcgaggtgccgtaaagcactaaatcggaaccctaaagggagcccccgatttagagcttgacggggaaagccggcgaacgtggcgagaaaggaagggaagaaagcgaaaggagcgggcgctagggcgctggcaagtgtagcggtcacgctgcgcgtaaccaccacacccgccgcgcttaatgcgccgctacagggcgcgtcccattcgccattcaggctgcgcaa

SEQ ID NO: 4 - DNA, 18 bp, Homo sapiens
  source 1..18: mol_type = genomic DNA
ggtcgtggcgacagcccg

SEQ ID NO: 5 - DNA, 1913 bp, adeno-associated virus 2
  source 1..1913: mol_type = genomic DNA
agtttcaggagcgccttaaagaagatacgtcttttgggggcaacctcggacgagcagtcttccaggcgaaaaagagggttcttgaacctctgggcctggttgaggaacctgttaagacggctccgggaaaaaagaggccggtagagcactctcctgtggagccagactcctcctcgggaaccggaaaggcgggccagcagcctgcaagaaaaagattgaattttggtcagactggagacgcagactcagtacctgacccccagcctctcggacagccaccagcagccccctctggtctgggaactaatacgatggctacaggcagtggcgcaccaatggcagacaataacgagggcgccgacggagtgggtaattcctcgggaaattggcattgcgattccacatggatgggcgacagagtcatcaccaccagcacccgaacctgggccctgcccacctacaacaaccacctctacaaacaaatttccagccaatcaggagcctcgaacgacaatcactactttggctacagcaccccttgggggtattttgacttcaacagattccactgccacttttcaccacgtgactggcaaagactcatcaacaacaactggggattccgacccaagagactcaacttcaagctctttaacattcaagtcaaagaggtcacgcagaatgacggtacgacgacgattgccaataaccttaccagcacggttcaggtgtttactgactcggagtaccagctcccgtacgtcctcggctcggcgcatcaaggatgcctcccgccgttcccagcagacgtcttcatggtgccacagtatggatacctcaccctgaacaacgggagtcaggcagtaggacgctcttcattttactgcctggagtactttccttctcagatgctgcgtaccggaaacaactttaccttcagctacacttttgaggacgttcctttccacagcagctacgctcacagccagagtctggaccgtctcatgaatcctctcatcgaccagtacctgtattacttgagcagaacaaacactccaagtggaaccaccacgcagtcaaggcttcagttttctcaggccggagcgagtgacattcgggaccagtctaggaactggcttcctggaccctgttaccgccagcagcgagtatcaaagacatctgcggataacaacaacagtgaatactcgtggactggagctaccaagtaccacctcaatggcagagactctctggtgaatccgggcccggccatggcaagccacaaggacgatgaagaaaagttttttcctcagagcggggttctcatctttgggaagcaaggctcagagaaaacaaatgtggacattgaaaaggtcatgattacagacgaagaggaaatcaggacaaccaatcccgtggctacggagcagtatggttctgtatctaccaacctccagagaggcaacagacaagcagctaccgcagatgtcaacacacaaggcgttcttccaggcatggtctggcaggacagagatgtgtaccttcaggggcccatctgggcaaagattccacacacggacggacattttcacccctctcccctcatgggtggattcggacttaaacaccctcctccacagattctcatcaagaacaccccggtacctgcgaatccttcgaccaccttcagtgcggcaaagtttgcttccttcatcacacagtactccacgggacaggtcagcgtggagatcgagtgggagctgcagaaggaaaacagcaaacgctggaatcccgaaattcagtacacttccaactacaacaagtctgttaatgtggactttactgtggacactaatggcgtgtattcagagcctcgccccattggcaccagatacctgactcgtaatctgtaa

SEQ ID NO: 6 - DNA, 7345 bp, synthetic construct
  source 1..7345: mol_type = other DNA
gacaggtttcccgactggaaagcgggcagtgagcgcaacgcaattaatgtgagttagctcactcattaggcaccccaggctttacactttatgcttccggctcgtatgttgtgtggaattgtgagcggataacaatttcacacaggaaacagctatgaccatgattacgccaagcgcgccgatatcgttaacgccccgcgccggccgctctagaactagtggatcccccggaagatcagaagttcctattccgaagttcctattctctagaaagtataggaacttctgatctgcgcagccgccatgccggggttttacgagattgtgattaaggtccccagcgaccttgacgagcatctgcccggcatttctgacagctttgtgaactgggtggccgagaaggaatgggagttgccgccagattctgacatggatctgaatctgattgagcaggcacccctgaccgtggccgagaagctgcagcgcgactttctgacggaatggcgccgtgtgagtaaggccccggaggcccttttctttgtgcaatttgagaagggagagagctacttccacatgcacgtgctcgtggaaaccaccggggtgaaatccatggttttgggacgtttcctgagtcagattcgcgaaaaactgattcagagaatttaccgcgggatcgagccgactttgccaaactggttcgcggtcacaaagaccagaaatggcgccggaggcgggaacaaggtggtggatgagtgctacatccccaattacttgctccccaaaacccagcctgagctccagtgggcgtggactaatatggaacagtatttaagcgcctgtttgaatctcacggagcgtaaacggttggtggcgcagcatctgacgcacgtgtcgcagacgcaggagcagaacaaagagaatcagaatcccaattctgatgcgccggtgatcagatcaaaaacttcagccaggtacatggagctggtcgggtggctcgtggacaaggggattacctcggagaagcagtggatccaggaggaccaggcctcatacatctccttcaatgcggcctccaactcgcggtcccaaatcaaggctgccttggacaatgcgggaaagattatgagcctgactaaaaccgcccccgactacctggtgggccagcagcccgtggaggacatttccagcaatcggatttataaaattttggaactaaacgggtacgatccccaatatgcggcttccgtctttctgggatgggccacgaaaaagttcggcaagaggaacaccatctggctgtttgggcctgcaactaccgggaagaccaacatcgcggaggccatagcccacactgtgcccttctacgggtgcgtaaactggaccaatgagaactttcccttcaacgactgtgtcgacaagatggtgatctggtgggaggaggggaagatgaccgccaaggtcgtggagtcggccaaagccattctcggaggaagcaaggtgcgcgtggaccagaaatgcaagtcctcggcccagatagacccgactcccgtgatcgtcacctccaacaccaacatgtgcgccgtgattgacgggaactcaacgaccttcgaacaccagcagccgttgcaagaccggatgttcaaatttgaactcacccgccgtctggatcatgactttgggaaggtcaccaagcaggaagtcaaagactttttccggtgggcaaaggatcacgtggttgaggtggagcatgaattctacgtcaaaaagggtggagccaagaaaagacccgcccccagtgacgcagatataagtgagcccaaacgggtgcgcgagtcagttgcgcagccatcgacgtcagacgcggaagcttcgatcaactacgcagacaggtaccaaaacaaatgttctcgtcacgtgggcatgaatctgatgctgtttccctgcagacaatgcgagagaatgaatcagaattcaaatatctgcttcactcacggacagaaagactgtttagagtgctttcccgtgtcagaatctcaacccgtttctgtcgtcaaaaaggcgtatcagaaactgtgctacattcatcatatcatgggaaaggtgccagacgcttgcactgcctgcgatctggtcaatgtggatttggatgactgcatctttgaacaataaatgatttaaatcaggtatggctgccgatggttatcttccagattggctcgaggacactctctctgaaggaataagacagtggtggaagctcaaacctggcccaccaccaccaaagcccgcagagcggcataaggacgacagcaggggtcttgtgcttcctgggtacaagtacctcggacccttcaacggactcgacaagggagagccggtcaacgaggcagacgccgcggccctcgagcacgacaaagcctacgaccggcagctcgacagcggagacaacccgtacctcaagtacaaccacgccgacgcggagtttcaggagcgccttaaagaagatacgtcttttgggggcaacctcggacgagcagtcttccaggcgaaaaagagggttcttgaacctctgggcctggttgaggaacctgttaagacggctccgggaaaaaagaggccggtagagcactctcctgtggagccagactcctcctcgggaaccggaaaggcgggccagcagcctgcaagaaaaagattgaattttggtcagactggagacgcagactcagtacctgacccccagcctctcggacagccaccagcagccccctctggtctgggaactaatacgatggctacaggcagtggcgcaccaatggcagacaataacgagggcgccgacggagtgggtaattcctcgggaaattggcattgcgattccacatggatgggcgacagagtcatcaccaccagcacccgaacctgggccctgcccacctacaacaaccacctctacaaacaaatttccagccaatcaggagcctcgaacgacaatcactactttggctacagcaccccttgggggtattttgacttcaacagattccactgccacttttcaccacgtgactggcaaagactcatcaacaacaactggggattccgacccaagagactcaacttcaagctctttaacattcaagtcaaagaggtcacgcagaatgacggtacgacgacgattgccaataaccttaccagcacggttcaggtgtttactgactcggagtaccagctcccgtacgtcctcggctcggcgcatcaaggatgcctcccgccgttcccagcagacgtcttcatggtgccacagtatggatacctcaccctgaacaacgggagtcaggcagtaggacgctcttcattttactgcctggagtactttccttctcagatgctgcgtaccggaaacaactttaccttcagctacacttttgaggacgttcctttccacagcagctacgctcacagccagagtctggaccgtctcatgaatcctctcatcgaccagtacctgtattacttgagcagaacaaacactccaagtggaggtcgtggcgacagcccgaccaccacgcagtcaaggcttcagttttctcaggccggagcgagtgacattcgggaccagtctaggaactggcttcctggaccctgttaccgccagcagcgagtatcaaagacatctgcggataacaacaacagtgaatactcgtggactggagctaccaagtaccacctcaatggcagagactctctggtgaatccgggcccggccatggcaagccacaaggacgatgaagaaaagttttttcctcagagcggggttctcatctttgggaagcaaggctcagagaaaacaaatgtggacattgaaaaggtcatgattacagacgaagaggaaatcaggacaaccaatcccgtggctacggagcagtatggttctgtatctaccaacctccagagaggcaacagacaagcagctaccgcagatgtcaacacacaaggcgttcttccaggcatggtctggcaggacagagatgtgtaccttcaggggcccatctgggcaaagattccacacacggacggacattttcacccctctcccctcatgggtggattcggacttaaacaccctcctccacagattctcatcaagaacaccccggtacctgcgaatccttcgaccaccttcagtgcggcaaagtttgcttccttcatcacacagtactccacgggacaggtcagcgtggagatcgagtgggagctgcagaaggaaaacagcaaacgctggaatcccgaaattcagtacacttccaactacaacaagtctgttaatgtggactttactgtggacactaatggcgtgtattcagagcctcgccccattggcaccagatacctgactcgtaatctgtaattgcttgttaatcaataaaccgtttaattcgtttcagttgaactttggtctctgcgtatttctttcttatctagtttccatggctacgtagataagtagcatggcgggttaatcattaactacagcccgggcgtttaaacagcgggcggaggggtggagtcgtgacgtgaattacgtcatagggttagggaggtcctgtattagaggtcacgtgagtgttttgcgacattttgcgacaccatgtggtctcgctgggggggggggcccgagtgagcacgcagggtctccattttgaagcgggaggtttgaacgagcgctggcgcgctcactggccgtcgttttacaacgtcgtgactgggaaaaccctggcgttacccaacttaatcgccttgcagcacatccccctttcgccagctggcgtaatagcgaagaggcccgcaccgatcgcccttcccaacagttgcgcagcctgaatggcgaatggaaattgtaagcgttaatattttgttaaaattcgcgttaaatttttgttaaatcagctcatttttttaaccaataggccgaaatcggcaaaatcccttataaatcaaaagaatagaccgagatagggttgagtgttgttccagtttggaacaagagtccactattaagaacgtggactccaacgtcaaagggcgaaaaaccgtctatcagggcgatggcccactacgtgaaccatcaccctaatcaagttttttggggtcgaggtgccgtaaagcactaaatcggaaccctaaagggagcccccgatttagagcttgacggggaaagccggcgaacgtggcgagaaaggaagggaagaaagcgaaaggagcgggcgctagggcgctggcaagtgtagcggtcacgctgcgcgtaaccaccacacccgccgcgcttaatgcgccgctacagggcgcgtcaggtggcacttttcggggaaatgtgcgcggaacccctatttgtttatttttctaaatacattcaaatatgtatccgctcatgagacaataaccctgataaatgcttcaataatattgaaaaaggaagagtatgagtattcaacatttccgtgtcgcccttattcccttttttgcggcattttgccttcctgtttttgctcacccagaaacgctggtgaaagtaaaagatgctgaagatcagttgggtgcacgagtgggttacatcgaactggatctcaacagcggtaagatccttgagagttttcgccccgaagaacgttttccaatgatgagcacttttaaagttctgctatgtggcgcggtattatcccgtattgacgccgggcaagagcaactcggtcgccgcatacactattctcagaatgacttggttgagtactcaccagtcacagaaaagcatcttacggatggcatgacagtaagagaattatgcagtgctgccataaccatgagtgataacactgcggccaacttacttctgacaacgatcggaggaccgaaggagctaaccgcttttttgcacaacatgggggatcatgtaactcgccttgatcgttgggaaccggagctgaatgaagccataccaaacgacgagcgtgacaccacgatgcctgtagcaatggcaacaacgttgcgcaaactattaactggcgaactacttactctagcttcccggcaacaattaatagactggatggaggcggataaagttgcaggaccacttctgcgctcggcccttccggctggctggtttattgctgataaatctggagccggtgagcgtgggtctcgcggtatcattgcagcactggggccagatggtaagccctcccgtatcgtagttatctacacgacggggagtcaggcaactatggatgaacgaaatagacagatcgctgagataggtgcctcactgattaagcattggtaactgtcagaccaagtttactcatatatactttagattgatttaaaacttcatttttaatttaaaaggatctaggtgaagatcctttttgataatctcatgaccaaaatcccttaacgtgagttttcgttccactgagcgtcagaccccgtagaaaagatcaaaggatcttcttgagatcctttttttctgcgcgtaatctgctgcttgcaaacaaaaaaaccaccgctaccagcggtggtttgtttgccggatcaagagctaccaactctttttccgaaggtaactggcttcagcagagcgcagataccaaatactgttcttctagtgtagccgtagttaggccaccacttcaagaactctgtagcaccgcctacatacctcgctctgctaatcctgttaccagtggctgctgccagtggcgataagtcgtgtcttaccgggttggactcaagacgatagttaccggataaggcgcagcggtcgggctgaacggggggttcgtgcacacagcccagcttggagcgaacgacctacaccgaactgagatacctacagcgtgagctatgagaaagcgccacgcttcccgaagggagaaaggcggacaggtatccggtaagcggcagggtcggaacaggagagcgcacgagggagcttccagggggaaacgcctggtatctttatagtcctgtcgggtttcgccacctctgacttgagcgtcgatttttgtgatgctcgtcaggggggcggagcctatggaaaaacgccagcaacgcggcctttttacggttcctggccttttgctggccttttgctcacatgttctttcctgcgttatcccctgattctgtggataaccgtattaccgcctttgagtgagctgataccgctcgccgcagccgaacgaccgagcgcagcgagtcagtgagcgaggaagcggaagagcgcccaatacgcaaaccgcctctccccgcgcgttggccgattcattaatgcagctggcac

SEQ ID NO: 7 - DNA, 7345 bp, synthetic construct
  source 1..7345: mol_type = other DNA
gacaggtttcccgactggaaagcgggcagtgagcgcaacgcaattaatgtgagttagctcactcattaggcaccccaggctttacactttatgcttccggctcgtatgttgtgtggaattgtgagcggataacaatttcacacaggaaacagctatgaccatgattacgccaagcgcgccgatatcgttaacgccccgcgccggccgctctagaactagtggatcccccggaagatcagaagttcctattccgaagttcctattctctagaaagtataggaacttctgatctgcgcagccgccatgccggggttttacgagattgtgattaaggtccccagcgaccttgacgagcatctgcccggcatttctgacagctttgtgaactgggtggccgagaaggaatgggagttgccgccagattctgacatggatctgaatctgattgagcaggcacccctgaccgtggccgagaagctgcagcgcgactttctgacggaatggcgccgtgtgagtaaggccccggaggcccttttctttgtgcaatttgagaagggagagagctacttccacatgcacgtgctcgtggaaaccaccggggtgaaatccatggttttgggacgtttcctgagtcagattcgcgaaaaactgattcagagaatttaccgcgggatcgagccgactttgccaaactggttcgcggtcacaaagaccagaaatggcgccggaggcgggaacaaggtggtggatgagtgctacatccccaattacttgctccccaaaacccagcctgagctccagtgggcgtggactaatatggaacagtatttaagcgcctgtttgaatctcacggagcgtaaacggttggtggcgcagcatctgacgcacgtgtcgcagacgcaggagcagaacaaagagaatcagaatcccaattctgatgcgccggtgatcagatcaaaaacttcagccaggtacatggagctggtcgggtggctcgtggacaaggggattacctcggagaagcagtggatccaggaggaccaggcctcatacatctccttcaatgcggcctccaactcgcggtcccaaatcaaggctgccttggacaatgcgggaaagattatgagcctgactaaaaccgcccccgactacctggtgggccagcagcccgtggaggacatttccagcaatcggatttataaaattttggaactaaacgggtacgatccccaatatgcggcttccgtctttctgggatgggccacgaaaaagttcggcaagaggaacaccatctggctgtttgggcctgcaactaccgggaagaccaacatcgcggaggccatagcccacactgtgcccttctacgggtgcgtaaactggaccaatgagaactttcccttcaacgactgtgtcgacaagatggtgatctggtgggaggaggggaagatgaccgccaaggtcgtggagtcggccaaagccattctcggaggaagcaaggtgcgcgtggaccagaaatgcaagtcctcggcccagatagacccgactcccgtgatcgtcacctccaacaccaacatgtgcgccgtgattgacgggaactcaacgaccttcgaacaccagcagccgttgcaagaccggatgttcaaatttgaactcacccgccgtctggatcatgactttgggaaggtcaccaagcaggaagtcaaagactttttccggtgggcaaaggatcacgtggttgaggtggagcatgaattctacgtcaaaaagggtggagccaagaaaagacccgcccccagtgacgcagatataagtgagcccaaacgggtgcgcgagtcagttgcgcagccatcgacgtcagacgcggaagcttcgatcaactacgcagacaggtaccaaaacaaatgttctcgtcacgtgggcatgaatctgatgctgtttccctgcagacaatgcgagagaatgaatcagaattcaaatatctgcttcactcacggacagaaagactgtttagagtgctttcccgtgtcagaatctcaacccgtttctgtcgtcaaaaaggcgtatcagaaactgtgctacattcatcatatcatgggaaaggtgccagacgcttgcactgcctgcgatctggtcaatgtggatttggatgactgcatctttgaacaataaatgatttaaatcaggtatggctgccgatggttatcttccagattggctcgaggacactctctctgaaggaataagacagtggtggaagctcaaacctggcccaccaccaccaaagcccgcagagcggcataaggacgacagcaggggtcttgtgcttcctgggtacaagtacctcggacccttcaacggactcgacaagggagagccggtcaacgaggcagacgccgcggccctcgagcacgacaaagcctacgaccggcagctcgacagcggagacaacccgtacctcaagtacaaccacgccgacgcggagtttcaggagcgccttaaagaagatacgtcttttgggggcaacctcggacgagcagtcttccaggcgaaaaagagggttcttgaacctctgggcctggttgaggaacctgttaagacggctccgggaaaaaagaggccggtagagcactctcctgtggagccagactcctcctcgggaaccggaaaggcgggccagcagcctgcaagaaaaagattgaattttggtcagactggagacgcagactcagtacctgacccccagcctctcggacagccaccagcagccccctctggtctgggaactaatacgatggctacaggcagtggcgcaccaatggcagacaataacgagggcgccgacggagtgggtaattcctcgggaaattggcattgcgattccacatggatgggcgacagagtcatcaccaccagcacccgaacctgggccctgcccacctacaacaaccacctctacaaacaaatttccagccaatcaggagcctcgaacgacaatcactactttggctacagcaccccttgggggtattttgacttcaacagattccactgccacttttcaccacgtgactggcaaagactcatcaacaacaactggggattccgacccaagagactcaacttcaagctctttaacattcaagtcaaagaggtcacgcagaatgacggtacgacgacgattgccaataaccttaccagcacggttcaggtgtttactgactcggagtaccagctcccgtacgtcctcggctcggcgcatcaaggatgcctcccgccgttcccagcagacgtcttcatggtgccacagtatggatacctcaccctgaacaacgggagtcaggcagtaggacgctcttcattttactgcctggagtactttccttctcagatgctgcgtaccggaaacaactttaccttcagctacacttttgaggacgttcctttccacagcagctacgctcacagccagagtctggaccgtctcatgaatcctctcatcgaccagtacctgtattacttgagcagaacaaacactccaagtggaaccaccacgcagtcaaggcttcagttttctcaggccggagcgagtgacattcgggaccagtctaggaactggcttcctggaccctgttaccgccagcagcgagtatcaaagacatctgcggataacaacaacagtgaatactcgtggactggagctaccaagtaccacctcaatggcagagactctctggtgaatccgggcccggccatggcaagccacaaggacgatgaagaaaagttttttcctcagagcggggttctcatctttgggaagcaaggctcagagaaaacaaatgtggacattgaaaaggtcatgattacagacgaagaggaaatcaggacaaccaatcccgtggctacggagcagtatggttctgtatctaccaacctccagagaggcaacagaggtcgtggcgacagcccgcaagcagctaccgcagatgtcaacacacaaggcgttcttccaggcatggtctggcaggacagagatgtgtaccttcaggggcccatctgggcaaagattccacacacggacggacattttcacccctctcccctcatgggtggattcggacttaaacaccctcctccacagattctcatcaagaacaccccggtacctgcgaatccttcgaccaccttcagtgcggcaaagtttgcttccttcatcacacagtactccacgggacaggtcagcgtggagatcgagtgggagctgcagaaggaaaacagcaaacgctggaatcccgaaattcagtacacttccaactacaacaagtctgttaatgtggactttactgtggacactaatggcgtgtattcagagcctcgccccattggcaccagatacctgactcgtaatctgtaattgcttgttaatcaataaaccgtttaattcgtttcagttgaactttggtctctgcgtatttctttcttatctagtttccatggctacgtagataagtagcatggcgggttaatcattaactacagcccgggcgtttaaacagcgggcggaggggtggagtcgtgacgtgaattacgtcatagggttagggaggtcctgtattagaggtcacgtgagtgttttgcgacattttgcgacaccatgtggtctcgctgggggggggggcccgagtgagcacgcagggtctccattttgaagcgggaggtttgaacgagcgctggcgcgctcactggccgtcgttttacaacgtcgtgactgggaaaaccctggcgttacccaacttaatcgccttgcagcacatccccctttcgccagctggcgtaatagcgaagaggcccgcaccgatcgcccttcccaacagttgcgcagcctgaatggcgaatggaaattgtaagcgttaatattttgttaaaattcgcgttaaatttttgttaaatcagctcatttttttaaccaataggccgaaatcggcaaaatcccttataaatcaaaagaatagaccgagatagggttgagtgttgttccagtttggaacaagagtccactattaagaacgtggactccaacgtcaaagggcgaaaaaccgtctatcagggcgatggcccactacgtgaaccatcaccctaatcaagttttttggggtcgaggtgccgtaaagcactaaatcggaaccctaaagggagcccccgatttagagcttgacggggaaagccggcgaacgtggcgagaaaggaagggaagaaagcgaaaggagcgggcgctagggcgctggcaagtgtagcggtcacgctgcgcgtaaccaccacacccgccgcgcttaatgcgccgctacagggcgcgtcaggtggcacttttcggggaaatgtgcgcggaacccctatttgtttatttttctaaatacattcaaatatgtatccgctcatgagacaataaccctgataaatgcttcaataatattgaaaaaggaagagtatgagtattcaacatttccgtgtcgcccttattcccttttttgcggcattttgccttcctgtttttgctcacccagaaacgctggtgaaagtaaaagatgctgaagatcagttgggtgcacgagtgggttacatcgaactggatctcaacagcggtaagatccttgagagttttcgccccgaagaacgttttccaatgatgagcacttttaaagttctgctatgtggcgcggtattatcccgtattgacgccgggcaagagcaactcggtcgccgcatacactattctcagaatgacttggttgagtactcaccagtcacagaaaagcatcttacggatggcatgacagtaagagaattatgcagtgctgccataaccatgagtgataacactgcggccaacttacttctgacaacgatcggaggaccgaaggagctaaccgcttttttgcacaacatgggggatcatgtaactcgccttgatcgttgggaaccggagctgaatgaagccataccaaacgacgagcgtgacaccacgatgcctgtagcaatggcaacaacgttgcgcaaactattaactggcgaactacttactctagcttcccggcaacaattaatagactggatggaggcggataaagttgcaggaccacttctgcgctcggcccttccggctggctggtttattgctgataaatctggagccggtgagcgtgggtctcgcggtatcattgcagcactggggccagatggtaagccctcccgtatcgtagttatctacacgacggggagtcaggcaactatggatgaacgaaatagacagatcgctgagataggtgcctcactgattaagcattggtaactgtcagaccaagtttactcatatatactttagattgatttaaaacttcatttttaatttaaaaggatctaggtgaagatcctttttgataatctcatgaccaaaatcccttaacgtgagttttcgttccactgagcgtcagaccccgtagaaaagatcaaaggatcttcttgagatcctttttttctgcgcgtaatctgctgcttgcaaacaaaaaaaccaccgctaccagcggtggtttgtttgccggatcaagagctaccaactctttttccgaaggtaactggcttcagcagagcgcagataccaaatactgttcttctagtgtagccgtagttaggccaccacttcaagaactctgtagcaccgcctacatacctcgctctgctaatcctgttaccagtggctgctgccagtggcgataagtcgtgtcttaccgggttggactcaagacgatagttaccggataaggcgcagcggtcgggctgaacggggggttcgtgcacacagcccagcttggagcgaacgacctacaccgaactgagatacctacagcgtgagctatgagaaagcgccacgcttcccgaagggagaaaggcggacaggtatccggtaagcggcagggtcggaacaggagagcgcacgagggagcttccagggggaaacgcctggtatctttatagtcctgtcgggtttcgccacctctgacttgagcgtcgatttttgtgatgctcgtcaggggggcggagcctatggaaaaacgccagcaacgcggcctttttacggttcctggccttttgctggccttttgctcacatgttctttcctgcgttatcccctgattctgtggataaccgtattaccgcctttgagtgagctgataccgctcgccgcagccgaacgaccgagcgcagcgagtcagtgagcgaggaagcggaagagcgcccaatacgcaaaccgcctctccccgcgcgttggccgattcattaatgcagctggcac

SEQ ID NO: 8 - DNA, 2211 bp, adeno-associated virus 6
  source 1..2211: mol_type = genomic DNA
atggctgccgatggttatcttccagattggctcgaggacaacctctctgagggcattcgcgagtggtgggacttgaaacctggagccccgaaacccaaagccaaccagcaaaagcaggacgacggccggggtctggtgcttcctggctacaagtacctcggacccttcaacggactcgacaagggggagcccgtcaacgcggcggatgcagcggccctcgagcacgacaaggcctacgaccagcagctcaaagcgggtgacaatccgtacctgcggtataaccacgccgacgccgagtttcaggagcgtctgcaagaagatacgtcttttgggggcaacctcgggcgagcagtcttccaggccaagaagagggttctcgaacctcttggtctggttgaggaaggtgctaagacggctcctggaaagaaacgtccggtagagcagtcgccacaagagccagactcctcctcgggcattggcaagacaggccagcagcccgctaaaaagagactcaattttggtcagactggcgactcagagtcagtccccgacccacaacctctcggagaacctccagcaacccccgctgctgtgggacctactacaatggcttcaggcggtggcgcaccaatggcagacaataacgaaggcgccgacggagtgggtaatgcctcaggaaattggcattgcgattccacatggctgggcgacagagtcatcaccaccagcacccgaacatgggccttgcccacctataacaaccacctctacaagcaaatctccagtgcttcaacgggggccagcaacgacaaccactacttcggctacagcaccccctgggggtattttgatttcaacagattccactgccatttctcaccacgtgactggcagcgactcatcaacaacaattggggattccggcccaagagactcaacttcaagctcttcaacatccaagtcaaggaggtcacgacgaatgatggcgtcacgaccatcgctaataaccttaccagcacggttcaagtcttctcggactcggagtaccagttgccgtacgtcctcggctctgcgcaccagggctgcctccctccgttcccggcggacgtgttcatgattccgcagtacggctacctaacgctcaacaatggcagccaggcagtgggacggtcatccttttactgcctggaatatttcccatcgcagatgctgagaacgggcaataactttaccttcagctacaccttcgaggacgtgcctttccacagcagctacgcgcacagccagagcctggaccggctgatgaatcctctcatcgaccagtacctgtattacctgaacagaactcagaatcagtccggaagtgcccaaaacaaggacttgctgtttagccgggggtctccagctggcatgtctgttcagcccaaaaactggctacctggaccctgttaccggcagcagcgcgtttctaaaacaaaaacagacaacaacaacagcaactttacctggactggtgcttcaaaatataaccttaatgggcgtgaatctataatcaaccctggcactgctatggcctcacacaaagacgacaaagacaagttctttcccatgagcggtgtcatgatttttggaaaggagagcgccggagcttcaaacactgcattggacaatgtcatgatcacagacgaagaggaaatcaaagccactaaccccgtggccaccgaaagatttgggactgtggcagtcaatctccagagcagcagcacagaccctgcgaccggagatgtgcatgttatgggagccttacctggaatggtgtggcaagacagagacgtatacctgcagggtcctatttgggccaaaattcctcacacggatggacactttcacccgtctcctctcatgggcggctttggacttaagcacccgcctcctcagatcctcatcaaaaacacgcctgttcctgcgaatcctccggcagagttttcggctacaaagtttgcttcattcatcacccagtattccacaggacaagtgagcgtggagattgaatgggagctgcagaaagaaaacagcaaacgctggaatcccgaagtgcagtatacatctaactatgcaaaatctgccaacgttgatttcactgtggacaacaatggactttatactgagcctcgccccattggcacccgttacctcacccgtcccctgtaa

SEQ ID NO: 9 - DNA, 7486 bp, synthetic construct
  source 1..7486: mol_type = other DNA
agggttgagtgttgttccagtttggaacaagagtccactattaaagaacgtggactccaacgtcaaagggcgaaaaaccgtctatcagggcgatggcccactacgtgaaccatcaccctaatcaagttttttggggtcgaggtgccgtaaagcactaaatcggaaccctaaagggagcccccgatttagagcttgacggggaaagccggcgaacgtggcgagaaaggaagggaagaaagcgaaaggagcgggcgctagggcgctggcaagtgtagcggtcacgctgcgcgtaaccaccacacccgccgcgcttaatgcgccgctacagggcgcgtccattcgccattcaggctgcgcaactgttgggaagggcgatcggtgcgggcctcttcgctattacgccagctggcgaaagggggatgtgctgcaaggcgattaagttgggtaacgccagggttttcccagtcacgacgttgtaaaacgacggccagtgaattgtaatacgactcactatagggcgaattcgagctcggtacccctagaggtcctgtattagaggtcacgtgagtgttttgcgacattttgcgacaccatgtggtcacgctgggtatttaagcccgagtgagcacgcagggtctccattttgaagcgggaggtttgaacgcgcagccaccacgccggggttttacgagattgtgattaaggtccccagcgaccttgacgagcatctgcccggcatttctgacagctttgtgaactgggtggccgagaaggaatgggagttgccgccagattctgacatggatctgaatctgattgagcaggcacccctgaccgtggccgagaagctgcagcgcgactttctgacggaatggcgccgtgtgagtaaggccccggaggcccttttctttgtgcaatttgagaagggagagagctacttccacatgcacgtgctcgtggaaaccaccggggtgaaatccatggttttgggacgtttcctgagtcagattcgcgaaaaactgattcagagaatttaccgcgggatcgagccgactttgccaaactggttcgcggtcacaaagaccagaaatggcgccggaggcgggaacaaggtggtggatgagtgctacatccccaattacttgctccccaaaacccagcctgagctccagtgggcgtggactaatatggaacagtatttaagcgcctgtttgaatctcacggagcgtaaacggttggtggcgcagcatctgacgcacgtgtcgcagacgcaggagcagaacaaagagaatcagaatcccaattctgatgcgccggtgatcagatcaaaaacttcagccaggtacatggagctggtcgggtggctcgtggacaaggggattacctcggagaagcagtggatccaggaggaccaggcctcatacatctccttcaatgcggcctccaactcgcggtcccaaatcaaggctgccttggacaatgcgggaaagattatgagcctgactaaaaccgcccccgactacctggtgggccagcagcccgtggaggacatttccagcaatcggatttataaaattttggaactaaacgggtacgatccccaatatgcggcttccgtctttctgggatgggccacgaaaaagttcggcaagaggaacaccatctggctgtttgggcctgcaactaccgggaagaccaacatcgcggaggccatagcccacactgtgcccttctacgggtgcgtaaactggaccaatgagaactttcccttcaacgactgtgtcgacaagatggtgatctggtgggaggagggcaagatgacggccaaggtcgtggagtccgccaaggccattctcggcggcagcaaggtgcgcgtggaccaaaagtgcaagtcgtccgcccagatcgatcccacccccgtgatcgtcacctccaacaccaacatgtgcgccgtgattgacgggaacagcaccaccttcgagcaccagcagccgttgcaggaccggatgttcaaatttgaactcacccgccgtctggagcatgactttggcaaggtgacaaagcaggaagtcaaagagttcttccgctgggcgcaggatcacgtgaccgaggtggcgcatgagttctacgtcagaaagggtggagccaacaagagacccgcccccgatgacgcggataaaagcgagcccaagcgggcctgcccctcagtcgcggatccatcgacgtcagacgcggaaggagctccggtggactttgccgacaggtaccaaaacaaatgttctcgtcacgcgggcatgcttcagatgctgtttccctgcaaaacatgcgagagaatgaatcagaatttcaacatttgcttcacgcacgggaccagagactgttcagaatgtttccccggcgtgtcagaatctcaaccggtcgtcagaaagaggacgtatcggaaactctgtgccattcatcatctgctggggcgggctcccgagattgcttgctcggcctgcgatctggtcaacgtggatctggatgactgtgtttctgagcaataaatgacttaaaccaggtatggctgccgatggttatcttccagattggctcgaggacaacctctctgagggcattcgcgagtggtgggacttgaaacctggagccccgaaacccaaagccaaccagcaaaagcaggacgacggccggggtctggtgcttcctggctacaagtacctcggacccttcaacggactcgacaagggggagcccgtcaacgcggcggatgcagcggccctcgagcacgacaaggcctacgaccagcagctcaaagcgggtgacaatccgtacctgcggtataaccacgccgacgccgagtttcaggagcgtctgcaagaagatacgtcttttgggggcaacctcgggcgagcagtcttccaggccaagaagagggttctcgaaccttttggtctggttgaggaaggtgctaagacggctcctggaaagaaacgtccggtagagcagtcgccacaagagccagactcctcctcgggcattggcaagacaggccagcagcccgctaaaaagagactcaattttggtcagactggcgactcagagtcagtccccgacccacaacctctcggagaacctccagcaacccccgctgctgtgggacctactacaatggcttcaggcggtggcgcaccaatggcagacaataacgaaggcgccgacggagtgggtaatgcctcaggaaattggcattgcgattccacatggctgggcgacagagtcatcaccaccagcacccgaacatgggccttgcccacctataacaaccacctctacaagcaaatctccagtgcttcaacgggggccagcaacgacaaccactacttcggctacagcaccccctgggggtattttgatttcaacagattccactgccatttctcaccacgtgactggcagcgactcatcaacaacaattggggattccggcccaagagactcaacttcaagctcttcaacatccaagtcaaggaggtcacgacgaatgatggcgtcacgaccatcgctaataaccttaccagcacggttcaagtcttctcggactcggagtaccagttgccgtacgtcctcggctctgcgcaccagggctgcctccctccgttcccggcggacgtgttcatgattccgcagtacggctacctaacgctcaacaatggcagccaggcagtgggacggtcatccttttactgcctggaatatttcccatcgcagatgctgagaacgggcaataactttaccttcagctacaccttcgaggacgtgcctttccacagcagctacgcgcacagccagagcctggaccggctgatgaatcctctcatcgaccagtacctgtattacctgaacagaactcagaatcagtccggaggtcgtggcgacagcccgagtgcccaaaacaaggacttgctgtttagccgggggtctccagctggcatgtctgttcagcccaaaaactggctacctggaccctgttaccggcagcagcgcgtttctaaaacaaaaacagacaacaacaacagcaactttacctggactggtgcttcaaaatataaccttaatgggcgtgaatctataatcaaccctggcactgctatggcctcacacaaagacgacaaagacaagttctttcccatgagcggtgtcatgatttttggaaaggagagcgccggagcttcaaacactgcattggacaatgtcatgatcacagacgaagaggaaatcaaagccactaaccccgtggccaccgaaagatttgggactgtggcagtcaatctccagagcagcagcacagaccctgcgaccggagatgtgcatgttatgggagccttacctggaatggtgtggcaagacagagacgtatacctgcagggtcctatttgggccaaaattcctcacacggatggacactttcacccgtctcctctcatgggcggctttggacttaagcacccgcctcctcagatcctcatcaaaaacacgcctgttcctgcgaatcctccggcagagttttcggctacaaagtttgcttcattcatcacccagtattccacaggacaagtgagcgtggagattgaatgggagctgcagaaagaaaacagcaaacgctggaatcccgaagtgcagtatacatctaactatgcaaaatctgccaacgttgatttcactgtggacaacaatggactttatactgagcctcgccccattggcacccgttacctcacccgtcccctgtaattgtctgttaatcaataaaccggttgattcgtttcagttgaactttggtctcgcggccgctcgataagcttttgttccctttagtgagggttaatttcgagcttggcgtaatcatggtcatagctgtttcctgtgtgaaattgttatccgctcacaattccacacaacatacgagccggaagcataaagtgtaaagcctggggtgcctaatgagtgagctaactcacattaattgcgttgcgctcactgcccgctttccagtcgggaaacctgtcgtgccagctgcattaatgaatcggccaacgcgcggggagaggcggtttgcgtattgggcgctcttccgcttcctcgctcactgactcgctgcgctcggtcgttcggctgcggcgagcggtatcagctcactcaaaggcggtaatacggttatccacagaatcaggggataacgcaggaaagaacatgtgagcaaaaggccagcaaaaggccaggaaccgtaaaaaggccgcgttgctggcgtttttccataggctccgcccccctgacgagcatcacaaaaatcgacgctcaagtcagaggtggcgaaacccgacaggactataaagataccaggcgtttccccctggaagctccctcgtgcgctctcctgttccgaccctgccgcttaccggatacctgtccgcctttctcccttcgggaagcgtggcgctttctcatagctcacgctgtaggtatctcagttcggtgtaggtcgttcgctccaagctgggctgtgtgcacgaaccccccgttcagcccgaccgctgcgccttatccggtaactatcgtcttgagtccaacccggtaagacacgacttatcgccactggcagcagccactggtaacaggattagcagagcgaggtatgtaggcggtgctacagagttcttgaagtggtggcctaactacggctacactagaagaacagtatttggtatctgcgctctgctgaagccagttaccttcggaaaaagagttggtagctcttgatccggcaaacaaaccaccgctggtagcggtggtttttttgtttgcaagcagcagattacgcgcagaaaaaaaggatctcaagaagatcctttgatcttttctacggggtctgacgctcagtggaacgaaaactcacgttaagggattttggtcatgagattatcaaaaaggatcttcacctagatccttttaaattaaaaatgaagttttaaatcaatctaaagtatatatgagtaaacttggtctgacagttaccaatgcttaatcagtgaggcacctatctcagcgatctgtctatttcgttcatccatagttgcctgactccccgtcgtgtagataactacgatacgggagggcttaccatctggccccagtgctgcaatgataccgcgagacccacgctcaccggctccagatttatcagcaataaaccagccagccggaagggccgagcgcagaagtggtcctgcaactttatccgcctccatccagtctattaattgttgccgggaagctagagtaagtagttcgccagttaatagtttgcgcaacgttgttgccattgctacaggcatcgtggtgtcacgctcgtcgtttggtatggcttcattcagctccggttcccaacgatcaaggcgagttacatgatcccccatgttgtgcaaaaaagcggttagctccttcggtcctccgatcgttgtcagaagtaagttggccgcagtgttatcactcatggttatggcagcactgcataattctcttactgtcatgccatccgtaagatgcttttctgtgactggtgagtactcaaccaagtcattctgagaatagtgtatgcggcgaccgagttgctcttgcccggcgtcaatacgggataataccgcgccacatagcagaactttaaaagtgctcatcattggaaaacgttcttcggggcgaaaactctcaaggatcttaccgctgttgagatccagttcgatgtaacccactcgtgcacccaactgatcttcagcatcttttactttcaccagcgtttctgggtgagcaaaaacaggaaggcaaaatgccgcaaaaaagggaataagggcgacacggaaatgttgaatactcatactcttcctttttcaatattattgaagcatttatcagggttattgtctcatgagcggatacatatttgaatgtatttagaaaaataaacaaataggggttccgcgcacatttccccgaaaagtgccacctgacgtctaagaaaccattattatcatgacattaacctataaaaataggcgtatcacgaggccctttcgtctcgcgcgtttcggtgatgacggtgaaaacctctgacacatgcagctcccggagacggtcacagcttgtctgtaagcggatgccgggagcagacaagcccgtcagggcgcgtcagcgggtgttggcgggtgtcggggctggcttaactatgcggcatcagagcagattgtactgagagtgcaccatatgcggtgtgaaataccgcacagatgcgtaaggagaaaataccgcatcaggaaattgtaagcgttaatattttgttaaaattcgcgttaaatttttgttaaatcagctcattttttaaccaataggccgaaatcggcaaaatcccttataaatcaaaagaatagaccgagat

SEQ ID NO: 10 - DNA, 7486 bp, synthetic construct
  source 1..7486: mol_type = other DNA
agggttgagtgttgttccagtttggaacaagagtccactattaaagaacgtggactccaacgtcaaagggcgaaaaaccgtctatcagggcgatggcccactacgtgaaccatcaccctaatcaagttttttggggtcgaggtgccgtaaagcactaaatcggaaccctaaagggagcccccgatttagagcttgacggggaaagccggcgaacgtggcgagaaaggaagggaagaaagcgaaaggagcgggcgctagggcgctggcaagtgtagcggtcacgctgcgcgtaaccaccacacccgccgcgcttaatgcgccgctacagggcgcgtccattcgccattcaggctgcgcaactgttgggaagggcgatcggtgcgggcctcttcgctattacgccagctggcgaaagggggatgtgctgcaaggcgattaagttgggtaacgccagggttttcccagtcacgacgttgtaaaacgacggccagtgaattgtaatacgactcactatagggcgaattcgagctcggtacccctagaggtcctgtattagaggtcacgtgagtgttttgcgacattttgcgacaccatgtggtcacgctgggtatttaagcccgagtgagcacgcagggtctccattttgaagcgggaggtttgaacgcgcagccaccacgccggggttttacgagattgtgattaaggtccccagcgaccttgacgagcatctgcccggcatttctgacagctttgtgaactgggtggccgagaaggaatgggagttgccgccagattctgacatggatctgaatctgattgagcaggcacccctgaccgtggccgagaagctgcagcgcgactttctgacggaatggcgccgtgtgagtaaggccccggaggcccttttctttgtgcaatttgagaagggagagagctacttccacatgcacgtgctcgtggaaaccaccggggtgaaatccatggttttgggacgtttcctgagtcagattcgcgaaaaactgattcagagaatttaccgcgggatcgagccgactttgccaaactggttcgcggtcacaaagaccagaaatggcgccggaggcgggaacaaggtggtggatgagtgctacatccccaattacttgctccccaaaacccagcctgagctccagtgggcgtggactaatatggaacagtatttaagcgcctgtttgaatctcacggagcgtaaacggttggtggcgcagcatctgacgcacgtgtcgcagacgcaggagcagaacaaagagaatcagaatcccaattctgatgcgccggtgatcagatcaaaaacttcagccaggtacatggagctggtcgggtggctcgtggacaaggggattacctcggagaagcagtggatccaggaggaccaggcctcatacatctccttcaatgcggcctccaactcgcggtcccaaatcaaggctgccttggacaatgcgggaaagattatgagcctgactaaaaccgcccccgactacctggtgggccagcagcccgtggaggacatttccagcaatcggatttataaaattttggaactaaacgggtacgatccccaatatgcggcttccgtctttctgggatgggccacgaaaaagttcggcaagaggaacaccatctggctgtttgggcctgcaactaccgggaagaccaacatcgcggaggccatagcccacactgtgcccttctacgggtgcgtaaactggaccaatgagaactttcccttcaacgactgtgtcgacaagatggtgatctggtgggaggagggcaagatgacggccaaggtcgtggagtccgccaaggccattctcggcggcagcaaggtgcgcgtggaccaaaagtgcaagtcgtccgcccagatcgatcccacccccgtgatcgtcacctccaacaccaacatgtgcgccgtgattgacgggaacagcaccaccttcgagcaccagcagccgttgcaggaccggatgttcaaatttgaactcacccgccgtctggagcatgactttggcaaggtgacaaagcaggaagtcaaagagttcttccgctgggcgcaggatcacgtgaccgaggtggcgcatgagttctacgtcagaaagggtggagccaacaagagacccgcccccgatgacgcggataaaagcgagcccaagcgggcctgcccctcagtcgcggatccatcgacgtcagacgcggaaggagctccggtggactttgccgacaggtaccaaaacaaatgttctcgtcacgcgggcatgcttcagatgctgtttccctgcaaaacatgcgagagaatgaatcagaatttcaacatttgcttcacgcacgggaccagagactgttcagaatgtttccccggcgtgtcagaatctcaaccggtcgtcagaaagaggacgtatcggaaactctgtgccattcatcatctgctggggcgggctcccgagattgcttgctcggcctgcgatctggtcaacgtggatctggatgactgtgtttctgagcaataaatgacttaaaccaggtatggctgccgatggttatcttccagattggctcgaggacaacctctctgagggcattcgcgagtggtgggacttgaaacctggagccccgaaacccaaagccaaccagcaaaagcaggacgacggccggggtctggtgcttcctggctacaagtacctcggacccttcaacggactcgacaagggggagcccgtcaacgcggcggatgcagcggccctcgagcacgacaaggcctacgaccagcagctcaaagcgggtgacaatccgtacctgcggtataaccacgccgacgccgagtttcaggagcgtctgcaagaagatacgtcttttgggggcaacctcgggcgagcagtcttccaggccaagaagagggttctcgaaccttttggtctggttgaggaaggtgctaagacggctcctggaaagaaacgtccggtagagcagtcgccacaagagccagactcctcctcgggcattggcaagacaggccagcagcccgctaaaaagagactcaattttggtcagactggcgactcagagtcagtccccgacccacaacctctcggagaacctccagcaacccccgctgctgtgggacctactacaatggcttcaggcggtggcgcaccaatggcagacaataacgaaggcgccgacggagtgggtaatgcctcaggaaattggcattgcgattccacatggctgggcgacagagtcatcaccaccagcacccgaacatgggccttgcccacctataacaaccacctctacaagcaaatctccagtgcttcaacgggggccagcaacgacaaccactacttcggctacagcaccccctgggggtattttgatttcaacagattccactgccatttctcaccacgtgactggcagcgactcatcaacaacaattggggattccggcccaagagactcaacttcaagctcttcaacatccaagtcaaggaggtcacgacgaatgatggcgtcacgaccatcgctaataaccttaccagcacggttcaagtcttctcggactcggagtaccagttgccgtacgtcctcggctctgcgcaccagggctgcctccctccgttcccggcggacgtgttcatgattccgcagtacggctacctaacgctcaacaatggcagccaggcagtgggacggtcatccttttactgcctggaatatttcccatcgcagatgctgagaacgggcaataactttaccttcagctacaccttcgaggacgtgcctttccacagcagctacgcgcacagccagagcctggaccggctgatgaatcctctcatcgaccagtacctgtattacctgaacagaactcagaatcagtccggaagtgcccaaaacaaggacttgctgtttagccgggggtctccagctggcatgtctgttcagcccaaaaactggctacctggaccctgttaccggcagcagcgcgtttctaaaacaaaaacagacaacaacaacagcaactttacctggactggtgcttcaaaatataaccttaatgggcgtgaatctataatcaaccctggcactgctatggcctcacacaaagacgacaaagacaagttctttcccatgagcggtgtcatgatttttggaaaggagagcgccggagcttcaaacactgcattggacaatgtcatgatcacagacgaagaggaaatcaaagccactaaccccgtggccaccgaaagatttgggactgtggcagtcaatctccagagcagcagcggtcgtggcgacagcccgacagaccctgcgaccggagatgtgcatgttatgggagccttacctggaatggtgtggcaagacagagacgtatacctgcagggtcctatttgggccaaaattcctcacacggatggacactttcacccgtctcctctcatgggcggctttggacttaagcacccgcctcctcagatcctcatcaaaaacacgcctgttcctgcgaatcctccggcagagttttcggctacaaagtttgcttcattcatcacccagtattccacaggacaagtgagcgtggagattgaatgggagctgcagaaagaaaacagcaaacgctggaatcccgaagtgcagtatacatctaactatgcaaaatctgccaacgttgatttcactgtggacaacaatggactttatactgagcctcgccccattggcacccgttacctcacccgtcccctgtaattgtctgttaatcaataaaccggttgattcgtttcagttgaactttggtctcgcggccgctcgataagcttttgttccctttagtgagggttaatttcgagcttggcgtaatcatggtcatagctgtttcctgtgtgaaattgttatccgctcacaattccacacaacatacgagccggaagcataaagtgtaaagcctggggtgcctaatgagtgagctaactcacattaattgcgttgcgctcactgcccgctttccagtcgggaaacctgtcgtgccagctgcattaatgaatcggccaacgcgcggggagaggcggtttgcgtattgggcgctcttccgcttcctcgctcactgactcgctgcgctcggtcgttcggctgcggcgagcggtatcagctcactcaaaggcggtaatacggttatccacagaatcaggggataacgcaggaaagaacatgtgagcaaaaggccagcaaaaggccaggaaccgtaaaaaggccgcgttgctggcgtttttccataggctccgcccccctgacgagcatcacaaaaatcgacgctcaagtcagaggtggcgaaacccgacaggactataaagataccaggcgtttccccctggaagctccctcgtgcgctctcctgttccgaccctgccgcttaccggatacctgtccgcctttctcccttcgggaagcgtggcgctttctcatagctcacgctgtaggtatctcagttcggtgtaggtcgttcgctccaagctgggctgtgtgcacgaaccccccgttcagcccgaccgctgcgccttatccggtaactatcgtcttgagtccaacccggtaagacacgacttatcgccactggcagcagccactggtaacaggattagcagagcgaggtatgtaggcggtgctacagagttcttgaagtggtggcctaactacggctacactagaagaacagtatttggtatctgcgctctgctgaagccagttaccttcggaaaaagagttggtagctcttgatccggcaaacaaaccaccgctggtagcggtggtttttttgtttgcaagcagcagattacgcgcagaaaaaaaggatctcaagaagatcctttgatcttttctacggggtctgacgctcagtggaacgaaaactcacgttaagggattttggtcatgagattatcaaaaaggatcttcacctagatccttttaaattaaaaatgaagttttaaatcaatctaaagtatatatgagtaaacttggtctgacagttaccaatgcttaatcagtgaggcacctatctcagcgatctgtctatttcgttcatccatagttgcctgactccccgtcgtgtagataactacgatacgggagggcttaccatctggccccagtgctgcaatgataccgcgagacccacgctcaccggctccagatttatcagcaataaaccagccagccggaagggccgagcgcagaagtggtcctgcaactttatccgcctccatccagtctattaattgttgccgggaagctagagtaagtagttcgccagttaatagtttgcgcaacgttgttgccattgctacaggcatcgtggtgtcacgctcgtcgtttggtatggcttcattcagctccggttcccaacgatcaaggcgagttacatgatcccccatgttgtgcaaaaaagcggttagctccttcggtcctccgatcgttgtcagaagtaagttggccgcagtgttatcactcatggttatggcagcactgcataattctcttactgtcatgccatccgtaagatgcttttctgtgactggtgagtactcaaccaagtcattctgagaatagtgtatgcggcgaccgagttgctcttgcccggcgtcaatacgggataataccgcgccacatagcagaactttaaaagtgctcatcattggaaaacgttcttcggggcgaaaactctcaaggatcttaccgctgttgagatccagttcgatgtaacccactcgtgcacccaactgatcttcagcatcttttactttcaccagcgtttctgggtgagcaaaaacaggaaggcaaaatgccgcaaaaaagggaataagggcgacacggaaatgttgaatactcatactcttcctttttcaatattattgaagcatttatcagggttattgtctcatgagcggatacatatttgaatgtatttagaaaaataaacaaataggggttccgcgcacatttccccgaaaagtgccacctgacgtctaagaaaccattattatcatgacattaacctataaaaataggcgtatcacgaggccctttcgtctcgcgcgtttcggtgatgacggtgaaaacctctgacacatgcagctcccggagacggtcacagcttgtctgtaagcggatgccgggagcagacaagcccgtcagggcgcgtcagcgggtgttggcgggtgtcggggctggcttaactatgcggcatcagagcagattgtactgagagtgcaccatatgcggtgtgaaataccgcacagatgcgtaaggagaaaataccgcatcaggaaattgtaagcgttaatattttgttaaaattcgcgttaaatttttgttaaatcagctcattttttaaccaataggccgaaatcggcaaaatcccttataaatcaaaagaatagaccgagat

SEQ ID NO: 11 - DNA, 2211 bp, adeno-associated virus 9
  source 1..2211: mol_type = genomic DNA
atggctgccgatggttatcttccagattggctcgaggacaaccttagtgaaggaattcgcgagtggtgggctttgaaacctggagcccctcaacccaaggcaaatcaacaacatcaagacaacgctcgaggtcttgtgcttccgggttacaaataccttggacccggcaacggactcgacaagggggagccggtcaacgcagcagacgcggcggccctcgagcacgacaaggcctacgaccagcagctcaaggccggagacaacccgtacctcaagtacaaccacgccgacgccgagttccaggagcggctcaaagaagatacgtcttttgggggcaacctcgggcgagcagtcttccaggccaaaaagaggcttcttgaacctcttggtctggttgaggaagcggctaagacggctcctggaaagaagaggcctgtagagcagtctcctcaggaaccggactcctccgcgggtattggcaaatcgggtgcacagcccgctaaaaagagactcaatttcggtcagactggcgacacagagtcagtcccagaccctcaaccaatcggagaacctcccgcagccccctcaggtgtgggatctcttacaatggcttcaggtggtggcgcaccagtggcagacaataacgaaggtgccgatggagtgggtagttcctcgggaaattggcattgcgattcccaatggctgggggacagagtcatcaccaccagcacccgaacctgggccctgcccacctacaacaatcacctctacaagcaaatctccaacagcacatctggaggatcttcaaatgacaacgcctacttcggctacagcaccccctgggggtattttgacttcaacagattccactgccacttctcaccacgtgactggcagcgactcatcaacaacaactggggattccggcctaagcgactcaacttcaagctcttcaacattcaggtcaaagaggttacggacaacaatggagtcaagaccatcgccaataaccttaccagcacggtccaggtcttcacggactcagactatcagctcccgtacgtgctcgggtcggctcacgagggctgcctcccgccgttcccagcggacgttttcatgattcctcagtacgggtatctgacgcttaatgatggaagccaggccgtgggtcgttcgtccttttactgcctggaatatttcccgtcgcaaatgctaagaacgggtaacaacttccagttcagctacgagtttgagaacgtacctttccatagcagctacgctcacagccaaagcctggaccgactaatgaatccactcatcgaccaatacttgtactatctctcaaagactattaacggttctggacagaatcaacaaacgctaaaattcagtgtggccggacccagcaacatggctgtccagggaagaaactacatacctggacccagctaccgacaacaacgtgtctcaaccactgtgactcaaaacaacaacagcgaatttgcttggcctggagcttcttcttgggctctcaatggacgtaatagcttgatgaatcctggacctgctatggccagccacaaagaaggagaggaccgtttctttcctttgtctggatctttaatttttggcaaacaaggaactggaagagacaacgtggatgcggacaaagtcatgataaccaacgaagaagaaattaaaactactaacccggtagcaacggagtcctatggacaagtggccacaaaccaccagagtgcccaagcacaggcgcagaccggctgggttcaaaaccaaggaatacttccgggtatggtttggcaggacagagatgtgtacctgcaaggacccatttgggccaaaattcctcacacggacggcaactttcacccttctccgctgatgggagggtttggaatgaagcacccgcctcctcagatcctcatcaaaaacacacctgtacctgcggatcctccaacggccttcaacaaggacaagctgaactctttcatcacccagtattctactggccaagtcagcgtggagatcgagtgggagctgcagaaggaaaacagcaagcgctggaacccggagatccagtacacttccaactattacaagtctaataatgttgaatttgctgttaatactgaaggtgtatatagtgaaccccgccccattggcaccagatacctgactcgtaatctgtaa

SEQ ID NO: 12 - DNA, 7348 bp, synthetic construct
  source 1..7348: mol_type = other DNA
tagggttgagtgttgttccagtttggaacaagagtccactattaaagaacgtggactccaacgtcaaagggcgaaaaaccgtctatcagggcgatggcccactacgtgaaccatcaccctaatcaagttttttggggtcgaggtgccgtaaagcactaaatcggaaccctaaagggagcccccgatttagagcttgacggggaaagccggcgaacgtggcgagaaaggaagggaagaaagcgaaaggagcgggcgctagggcgctggcaagtgtagcggtcacgctgcgcgtaaccaccacacccgccgcgcttaatgcgccgctacagggcgcgtcccattcgccattcaggctgcgcaactgttgggaagggcgatcggtgcgggcctcttcgctattacgccagctggcgaaagggggatgtgctgcaaggcgattaagttgggtaacgccagggttttcccagtcacgacgttgtaaaacgacggccagtgagcgcgcgtaatacgactcactatagggcgaattgggtaccgggccccccctcgatcgaggtcgacggtatcgggggagctcgcagggtctccattttgaagcgggaggtttgaacgcgcagccgccatgccggggttttacgagattgtgattaaggtccccagcgaccttgacgagcatctgcccggcatttctgacagctttgtgaactgggtggccgagaaggaatgggagttgccgccagattctgacatggatctgaatctgattgagcaggcacccctgaccgtggccgagaagctgcagcgcgactttctgacggaatggcgccgtgtgagtaaggccccggaggctcttttctttgtgcaatttgagaagggagagagctacttccacatgcacgtgctcgtggaaaccaccggggtgaaatccatggttttgggacgtttcctgagtcagattcgcgaaaaactgattcagagaatttaccgcgggatcgagccgactttgccaaactggttcgcggtcacaaagaccagaaatggcgccggaggcgggaacaaggtggtggatgagtgctacatccccaattacttgctccccaaaacccagcctgagctccagtgggcgtggactaatatggaacagtatttaagcgcctgtttgaatctcacggagcgtaaacggttggtggcgcagcatctgacgcacgtgtcgcagacgcaggagcagaacaaagagaatcagaatcccaattctgatgcgccggtgatcagatcaaaaacttcagccaggtacatggagctggtcgggtggctcgtggacaaggggattacctcggagaagcagtggatccaggaggaccaggcctcatacatctccttcaatgcggcctccaactcgcggtcccaaatcaaggctgccttggacaatgcgggaaagattatgagcctgactaaaaccgcccccgactacctggtgggccagcagcccgtggaggacatttccagcaatcggatttataaaattttggaactaaacgggtacgatccccaatatgcggcttccgtctttctgggatgggccacgaaaaagttcggcaagaggaacaccatctggctgtttgggcctgcaactaccgggaagaccaacatcgcggaggccatagcccacactgtgcccttctacgggtgcgtaaactggaccaatgagaactttcccttcaacgactgtgtcgacaagatggtgatctggtgggaggaggggaagatgaccgccaaggtcgtggagtcggccaaagccattctcggaggaagcaaggtgcgcgtggaccagaaatgcaagtcctcggcccagatagacccgactcccgtgatcgtcacctccaacaccaacatgtgcgccgtgattgacgggaactcaacgaccttcgaacaccagcagccgttgcaagaccggatgttcaaatttgaactcacccgccgtctggatcatgactttgggaaggtcaccaagcaggaagtcaaagactttttccggtgggcaaaggatcacgtggttgaggtggagcatgaattctacgtcaaaaagggtggagccaagaaaagacccgcccccagtgacgcagatataagtgagcccaaacgggtgcgcgagtcagttgcgcagccatcgacgtcagacgcggaagcttcgatcaactacgcagacaggtaccaaaacaaatgttctcgtcacgtgggcatgaatctgatgctgtttccctgcagacaatgcgagagaatgaatcagaattcaaatatctgcttcactcacggacagaaagactgtttagagtgctttcccgtgtcagaatctcaacccgtttctgtcgtcaaaaaggcgtatcagaaactgtgctacattcatcatatcatgggaaaggtgccagacgcttgcactgcctgcgatctggtcaatgtggatttggatgactgcatctttgaacaataaatgatttaaatcaggtatggctgccgatggttatcttccagattggctcgaggacaaccttagtgaaggaattcgcgagtggtgggctttgaaacctggagcccctcaacccaaggcaaatcaacaacatcaagacaacgctcgaggtcttgtgcttccgggttacaaataccttggacccggcaacggactcgacaagggggagccggtcaacgcagcagacgcggcggccctcgagcacgacaaggcctacgaccagcagctcaaggccggagacaacccgtacctcaagtacaaccacgccgacgccgagttccaggagcggctcaaagaagatacgtcttttgggggcaacctcgggcgagcagtcttccaggccaaaaagaggcttcttgaacctcttggtctggttgaggaagcggctaagacggctcctggaaagaagaggcctgtagagcagtctcctcaggaaccggactcctccgcgggtattggcaaatcgggtgcacagcccgctaaaaagagactcaatttcggtcagactggcgacacagagtcagtcccagaccctcaaccaatcggagaacctcccgcagccccctcaggtgtgggatctcttacaatggcttcaggtggtggcgcaccagtggcagacaataacgaaggtgccgatggagtgggtagttcctcgggaaattggcattgcgattcccaatggctgggggacagagtcatcaccaccagcacccgaacctgggccctgcccacctacaacaatcacctctacaagcaaatctccaacagcacatctggaggatcttcaaatgacaacgcctacttcggctacagcaccccctgggggtattttgacttcaacagattccactgccacttctcaccacgtgactggcagcgactcatcaacaacaactggggattccggcctaagcgactcaacttcaagctcttcaacattcaggtcaaagaggttacggacaacaatggagtcaagaccatcgccaataaccttaccagcacggtccaggtcttcacggactcagactatcagctcccgtacgtgctcgggtcggctcacgagggctgcctcccgccgttcccagcggacgttttcatgattcctcagtacgggtatctgacgcttaatgatggaagccaggccgtgggtcgttcgtccttttactgcctggaatatttcccgtcgcaaatgctaagaacgggtaacaacttccagttcagctacgagtttgagaacgtacctttccatagcagctacgctcacagccaaagcctggaccgactaatgaatccactcatcgaccaatacttgtactatctctcaaagactattaacggttctggaggtcgtggcgacagcccgcagaatcaacaaacgctaaaattcagtgtggccggacccagcaacatggctgtccagggaagaaactacatacctggacccagctaccgacaacaacgtgtctcaaccactgtgactcaaaacaacaacagcgaatttgcttggcctggagcttcttcttgggctctcaatggacgtaatagcttgatgaatcctggacctgctatggccagccacaaagaaggagaggaccgtttctttcctttgtctggatctttaatttttggcaaacaaggaactggaagagacaacgtggatgcggacaaagtcatgataaccaacgaagaagaaattaaaactactaacccggtagcaacggagtcctatggacaagtggccacaaaccaccagagtgcccaagcacaggcgcagaccggctgggttcaaaaccaaggaatacttccgggtatggtttggcaggacagagatgtgtacctgcaaggacccatttgggccaaaattcctcacacggacggcaactttcacccttctccgctgatgggagggtttggaatgaagcacccgcctcctcagatcctcatcaaaaacacacctgtacctgcggatcctccaacggccttcaacaaggacaagctgaactctttcatcacccagtattctactggccaagtcagcgtggagatcgagtgggagctgcagaaggaaaacagcaagcgctggaacccggagatccagtacacttccaactattacaagtctaataatgttgaatttgctgttaatactgaaggtgtatatagtgaaccccgccccattggcaccagatacctgactcgtaatctgtaattgcttgttaatcaataaaccgtttaattcgtttcagttgaactttggtctctgcgaagggcgaattcgtttaaacctgcaggactagaggtcctgtattagaggtcacgtgagtgttttgcgacattttgcgacaccatgtggtcacgctgggtatttaagcccgagtgagcacgcagggtctccattttgaagcgggaggtttgaacgcgcagccgccaagccgaattctgcagatatccatcacactggcggccgctcgactagagcggccgccaccgcggtggagctccagcttttgttccctttagtgagggttaattgcgcgcttggcgtaatcatggtcatagctgtttcctgtgtgaaattgttatccgctcacaattccacacaacatacgagccggaagcataaagtgtaaagcctggggtgcctaatgagtgagctaactcacattaattgcgttgcgctcactgcccgctttccagtcgggaaacctgtcgtgccagctgcattaatgaatcggccaacgcgcggggagaggcggtttgcgtattgggcgctcttccgcttcctcgctcactgactcgctgcgctcggtcgttcggctgcggcgagcggtatcagctcactcaaaggcggtaatacggttatccacagaatcaggggataacgcaggaaagaacatgtgagcaaaaggccagcaaaaggccaggaaccgtaaaaaggccgcgttgctggcgtttttccataggctccgcccccctgacgagcatcacaaaaatcgacgctcaagtcagaggtggcgaaacccgacaggactataaagataccaggcgtttccccctggaagctccctcgtgcgctctcctgttccgaccctgccgcttaccggatacctgtccgcctttctcccttcgggaagcgtggcgctttctcatagctcacgctgtaggtatctcagttcggtgtaggtcgttcgctccaagctgggctgtgtgcacgaaccccccgttcagcccgaccgctgcgccttatccggtaactatcgtcttgagtccaacccggtaagacacgacttatcgccactggcagcagccactggtaacaggattagcagagcgaggtatgtaggcggtgctacagagttcttgaagtggtggcctaactacggctacactagaagaacagtatttggtatctgcgctctgctgaagccagttaccttcggaaaaagagttggtagctcttgatccggcaaacaaaccaccgctggtagcggtggtttttttgtttgcaagcagcagattacgcgcagaaaaaaaggatctcaagaagatcctttgatcttttctacggggtctgacgctcagtggaacgaaaactcacgttaagggattttggtcatgagattatcaaaaaggatcttcacctagatccttttaaattaaaaatgaagttttaaatcaatctaaagtatatatgagtaaacttggtctgacagttaccaatgcttaatcagtgaggcacctatctcagcgatctgtctatttcgttcatccatagttgcctgactccccgtcgtgtagataactacgatacgggagggcttaccatctggccccagtgctgcaatgataccgcgagacccacgctcaccggctccagatttatcagcaataaaccagccagccggaagggccgagcgcagaagtggtcctgcaactttatccgcctccatccagtctattaattgttgccgggaagctagagtaagtagttcgccagttaatagtttgcgcaacgttgttgccattgctacaggcatcgtggtgtcacgctcgtcgtttggtatggcttcattcagctccggttcccaacgatcaaggcgagttacatgatcccccatgttgtgcaaaaaagcggttagctccttcggtcctccgatcgttgtcagaagtaagttggccgcagtgttatcactcatggttatggcagcactgcataattctcttactgtcatgccatccgtaagatgcttttctgtgactggtgagtactcaaccaagtcattctgagaatagtgtatgcggcgaccgagttgctcttgcccggcgtcaatacgggataataccgcgccacatagcagaactttaaaagtgctcatcattggaaaacgttcttcggggcgaaaactctcaaggatcttaccgctgttgagatccagttcgatgtaacccactcgtgcacccaactgatcttcagcatcttttactttcaccagcgtttctgggtgagcaaaaacaggaaggcaaaatgccgcaaaaaagggaataagggcgacacggaaatgttgaatactcatactcttcctttttcaatattattgaagcatttatcagggttattgtctcatgagcggatacatatttgaatgtatttagaaaaataaacaaataggggttccgcgcacatttccccgaaaagtgccacctaaattgtaagcgttaatattttgttaaaattcgcgttaaatttttgttaaatcagctcattttttaaccaataggccgaaatcggcaaaatcccttataaatcaaaagaatagaccgaga

SEQ ID NO: 13 - DNA, 7348 bp, synthetic construct
  source 1..7348: mol_type = other DNA
ctgttgggaagggcgatcggtgcgggcctcttcgctattacgccagctggcgaaagggggatgtgctgcaaggcgattaagttgggtaacgccagggttttcccagtcacgacgttgtaaaacgacggccagtgagcgcgcgtaatacgactcactatagggcgaattgggtaccgggccccccctcgatcgaggtcgacggtatcgggggagctcgcagggtctccattttgaagcgggaggtttgaacgcgcagccgccatgccggggttttacgagattgtgattaaggtccccagcgaccttgacgagcatctgcccggcatttctgacagctttgtgaactgggtggccgagaaggaatgggagttgccgccagattctgacatggatctgaatctgattgagcaggcacccctgaccgtggccgagaagctgcagcgcgactttctgacggaatggcgccgtgtgagtaaggccccggaggctcttttctttgtgcaatttgagaagggagagagctacttccacatgcacgtgctcgtggaaaccaccggggtgaaatccatggttttgggacgtttcctgagtcagattcgcgaaaaactgattcagagaatttaccgcgggatcgagccgactttgccaaactggttcgcggtcacaaagaccagaaatggcgccggaggcgggaacaaggtggtggatgagtgctacatccccaattacttgctccccaaaacccagcctgagctccagtgggcgtggactaatatggaacagtatttaagcgcctgtttgaatctcacggagcgtaaacggttggtggcgcagcatctgacgcacgtgtcgcagacgcaggagcagaacaaagagaatcagaatcccaattctgatgcgccggtgatcagatcaaaaacttcagccaggtacatggagctggtcgggtggctcgtggacaaggggattacctcggagaagcagtggatccaggaggaccaggcctcatacatctccttcaatgcggcctccaactcgcggtcccaaatcaaggctgccttggacaatgcgggaaagattatgagcctgactaaaaccgcccccgactacctggtgggccagcagcccgtggaggacatttccagcaatcggatttataaaattttggaactaaacgggtacgatccccaatatgcggcttccgtctttctgggatgggccacgaaaaagttcggcaagaggaacaccatctggctgtttgggcctgcaactaccgggaagaccaacatcgcggaggccatagcccacactgtgcccttctacgggtgcgtaaactggaccaatgagaactttcccttcaacgactgtgtcgacaagatggtgatctggtgggaggaggggaagatgaccgccaaggtcgtggagtcggccaaagccattctcggaggaagcaaggtgcgcgtggaccagaaatgcaagtcctcggcccagatagacccgactcccgtgatcgtcacctccaacaccaacatgtgcgccgtgattgacgggaactcaacgaccttcgaacaccagcagccgttgcaagaccggatgttcaaatttgaactcacccgccgtctggatcatgactttgggaaggtcaccaagcaggaagtcaaagactttttccggtgggcaaaggatcacgtggttgaggtggagcatgaattctacgtcaaaaagggtggagccaagaaaagacccgcccccagtgacgcagatataagtgagcccaaacgggtgcgcgagtcagttgcgcagccatcgacgtcagacgcggaagcttcgatcaactacgcggacaggtaccaaaacaaatgttctcgtcacgtgggcatgaatctgatgctgtttccctgcagacaatgcgagagactgaatcagaattcaaatatctgcttcactcacggtgtcaaagactgtttagagtgctttcccgtgtcagaatctcaacccgtttctgtcgtcaaaaaggcgtatcagaaactgtgctacattcatcacatcatgggaaaggtgccagacgcttgcactgcttgcgacctggtcaatgtggacttggatgactgtgtttctgaacaataaatgacttaaaccaggtatggctgccgatggttatcttccagattggctcgaggacaaccttagtgaaggaattcgcgagtggtgggctttgaaacctggagcccctcaacccaaggcaaatcaacaacatcaagacaacgctcgaggtcttgtgcttccgggttacaaataccttggacccggcaacggactcgacaagggggagccggtcaacgcagcagacgcggcggccctcgagcacgacaaggcctacgaccagcagctcaaggccggagacaacccgtacctcaagtacaaccacgccgacgccgagttccaggagcggctcaaagaagatacgtcttttgggggcaacctcgggcgagcagtcttccaggccaaaaagaggcttcttgaacctcttggtctggttgaggaagcggctaagacggctcctggaaagaagaggcctgtagagcagtctcctcaggaaccggactcctccgcgggtattggcaaatcgggtgcacagcccgctaaaaagagactcaatttcggtcagactggcgacacagagtcagtcccagaccctcaaccaatcggagaacctcccgcagccccctcaggtgtgggatctcttacaatggcttcaggtggtggcgcaccagtggcagacaataacgaaggtgccgatggagtgggtagttcctcgggaaattggcattgcgattcccaatggctgggggacagagtcatcaccaccagcacccgaacctgggccctgcccacctacaacaatcacctctacaagcaaatctccaacagcacatctggaggatcttcaaatgacaacgcctacttcggctacagcaccccctgggggtattttgacttcaacagattccactgccacttctcaccacgtgactggcagcgactcatcaacaacaactggggattccggcctaagcgactcaacttcaagctcttcaacattcaggtcaaagaggttacggacaacaatggagtcaagaccatcgccaataaccttaccagcacggtccaggtcttcacggactcagactatcagctcccgtacgtgctcgggtcggctcacgagggctgcctcccgccgttcccagcggacgttttcatgattcctcagtacgggtatctgacgcttaatgatggaagccaggccgtgggtcgttcgtccttttactgcctggaatatttcccgtcgcaaatgctaagaacgggtaacaacttccagttcagctacgagtttgagaacgtacctttccatagcagctacgctcacagccaaagcctggaccgactaatgaatccactcatcgaccaatacttgtactatctctcaaagactattaacggttctggacagaatcaacaaacgctaaaattcagtgtggccggacccagcaacatggctgtccagggaagaaactacatacctggacccagctaccgacaacaacgtgtctcaaccactgtgactcaaaacaacaacagcgaatttgcttggcctggagcttcttcttgggctctcaatggacgtaatagcttgatgaatcctggacctgctatggccagccacaaagaaggagaggaccgtttctttcctttgtctggatctttaatttttggcaaacaaggaactggaagagacaacgtggatgcggacaaagtcatgataaccaacgaagaagaaattaaaactactaacccggtagcaacggagtcctatggacaagtggccacaaaccaccagagtgcccaaggtcgtggcgacagcccggcacaggcgcagaccggctgggttcaaaaccaaggaatacttccgggtatggtttggcaggacagagatgtgtacctgcaaggacccatttgggccaaaattcctcacacggacggcaactttcacccttctccgctgatgggagggtttggaatgaagcacccgcctcctcagatcctcatcaaaaacacacctgtacctgcggatcctccaacggccttcaacaaggacaagctgaactctttcatcacccagtattctactggccaagtcagcgtggagatcgagtgggagctgcagaaggaaaacagcaagcgctggaacccggagatccagtacacttccaactattacaagtctaataatgttgaatttgctgttaatactgaaggtgtatatagtgaaccccgccccattggcaccagatacctgactcgtaatctgtaattgcttgttaatcaataaaccgtttaattcgtttcagttgaactttggtctctgcgaagggcgaattcgtttaaacctgcaggactagaggtcctgtattagaggtcacgtgagtgttttgcgacattttgcgacaccatgtggtcacgctgggtatttaagcccgagtgagcacgcagggtctccattttgaagcgggaggtttgaacgcgcagccgccaagccgaattctgcagatatccatcacactggcggccgctcgactagagcggccgccaccgcggtggagctccagcttttgttccctttagtgagggttaattgcgcgcttggcgtaatcatggtcatagctgtttcctgtgtgaaattgttatccgctcacaattccacacaacatacgagccggaagcataaagtgtaaagcctggggtgcctaatgagtgagctaactcacattaattgcgttgcgctcactgcccgctttccagtcgggaaacctgtcgtgccagctgcattaatgaatcggccaacgcgcggggagaggcggtttgcgtattgggcgctcttccgcttcctcgctcactgactcgctgcgctcggtcgttcggctgcggcgagcggtatcagctcactcaaaggcggtaatacggttatccacagaatcaggggataacgcaggaaagaacatgtgagcaaaaggccagcaaaaggccaggaaccgtaaaaaggccgcgttgctggcgtttttccataggctccgcccccctgacgagcatcacaaaaatcgacgctcaagtcagaggtggcgaaacccgacaggactataaagataccaggcgtttccccctggaagctccctcgtgcgctctcctgttccgaccctgccgcttaccggatacctgtccgcctttctcccttcgggaagcgtggcgctttctcatagctcacgctgtaggtatctcagttcggtgtaggtcgttcgctccaagctgggctgtgtgcacgaaccccccgttcagcccgaccgctgcgccttatccggtaactatcgtcttgagtccaacccggtaagacacgacttatcgccactggcagcagccactggtaacaggattagcagagcgaggtatgtaggcggtgctacagagttcttgaagtggtggcctaactacggctacactagaagaacagtatttggtatctgcgctctgctgaagccagttaccttcggaaaaagagttggtagctcttgatccggcaaacaaaccaccgctggtagcggtggtttttttgtttgcaagcagcagattacgcgcagaaaaaaaggatctcaagaagatcctttgatcttttctacggggtctgacgctcagtggaacgaaaactcacgttaagggattttggtcatgagattatcaaaaaggatcttcacctagatccttttaaattaaaaatgaagttttaaatcaatctaaagtatatatgagtaaacttggtctgacagttaccaatgcttaatcagtgaggcacctatctcagcgatctgtctatttcgttcatccatagttgcctgactccccgtcgtgtagataactacgatacgggagggcttaccatctggccccagtgctgcaatgataccgcgagacccacgctcaccggctccagatttatcagcaataaaccagccagccggaagggccgagcgcagaagtggtcctgcaactttatccgcctccatccagtctattaattgttgccgggaagctagagtaagtagttcgccagttaatagtttgcgcaacgttgttgccattgctacaggcatcgtggtgtcacgctcgtcgtttggtatggcttcattcagctccggttcccaacgatcaaggcgagttacatgatcccccatgttgtgcaaaaaagcggttagctccttcggtcctccgatcgttgtcagaagtaagttggccgcagtgttatcactcatggttatggcagcactgcataattctcttactgtcatgccatccgtaagatgcttttctgtgactggtgagtactcaaccaagtcattctgagaatagtgtatgcggcgaccgagttgctcttgcccggcgtcaatacgggataataccgcgccacatagcagaactttaaaagtgctcatcattggaaaacgttcttcggggcgaaaactctcaaggatcttaccgctgttgagatccagttcgatgtaacccactcgtgcacccaactgatcttcagcatcttttactttcaccagcgtttctgggtgagcaaaaacaggaaggcaaaatgccgcaaaaaagggaataagggcgacacggaaatgttgaatactcatactcttcctttttcaatattattgaagcatttatcagggttattgtctcatgagcggatacatatttgaatgtatttagaaaaataaacaaataggggttccgcgcacatttccccgaaaagtgccacctaaattgtaagcgttaatattttgttaaaattcgcgttaaatttttgttaaatcagctcattttttaaccaataggccgaaatcggcaaaatcccttataaatcaaaagaatagaccgagatagggttgagtgttgttccagtttggaacaagagtccactattaaagaacgtggactccaacgtcaaagggcgaaaaaccgtctatcagggcgatggcccactacgtgaaccatcaccctaatcaagttttttggggtcgaggtgccgtaaagcactaaatcggaaccctaaagggagcccccgatttagagcttgacggggaaagccggcgaacgtggcgagaaaggaagggaagaaagcgaaaggagcgggcgctagggcgctggcaagtgtagcggtcacgctgcgcgtaaccaccacacccgccgcgcttaatgcgccgctacagggcgcgtcccattcgccattcaggctgcgcaa

SEQ ID NO: 14 - protein, 735 aa, adeno-associated virus 2 [sequence omitted]

SEQ ID NO: 15 - protein, 598 aa, adeno-associated virus 2
TAPGKKRPVEHSPVEPDSSSGTGKAGQQPARKRLNFGQTGDADSVPDPQPLGQPPAAPSGLGTNTMATGSGAPMADNNEGADGVGNSSGNWHCDSTWMGDRVITTSTRTWALPTYNNHLYKQISSQSGASNDNHYFGYSTPWGYFDFNRFHCHFSPRDWQRLINNNWGFRPKRLNFKLFNIQVKEVTQNDGTTTIANNLTSTVQVFTDSEYQLPYVLGSAHQGCLPPFPADVFMVPQYGYLTLNNGSQAVGRSSFYCLEYFPSQMLRTGNNFTFSYTFEDVPFHSSYAHSQSLDRLMNPLIDQYLYYLSRTNTPSGTTTQSRLQFSQAGASDIRDQSRNWLPGPCYRQQRVSKTSADNNNSEYSWTGATKYHLNGRDSLVNPGPAMASHKDDEEKFFPQSGVLIFGKQGSEKTNVDIEKVMITDEEEIRTTNPVATEQYGSVSTNLQRGNRQAATADVNTQGVLPGMVWQDRDVYLQGPIWAKIPHTDGHFHPSPLMGGFGLKHPPPQILIKNTPVPANPSTTFSAAKFASFITQYSTGQVSVEIEWELQKENSKRWNPEIQYTSNYNKSVNVDFTVDTNGVYSEPRPIGTRYLTRNL

SEQ ID NO: 16 - protein, 533 aa, adeno-associated virus 2
MATGSGAPMADNNEGADGVGNSSGNWHCDSTWMGDRVITTSTRTWALPTYNNHLYKQISSQSGASNDNHYFGYSTPWGYFDFNRFHCHFSPRDWQRLINNNWGFRPKRLNFKLFNIQVKEVTQNDGTTTIANNLTSTVQVFTDSEYQLPYVLGSAHQGCLPPFPADVFMVPQYGYLTLNNGSQAVGRSSFYCLEYFPSQMLRTGNNFTFSYTFEDVPFHSSYAHSQSLDRLMNPLIDQYLYYLSRTNTPSGTTTQSRLQFSQAGASDIRDQSRNWLPGPCYRQQRVSKTSADNNNSEYSWTGATKYHLNGRDSLVNPGPAMASHKDDEEKFFPQSGVLIFGKQGSEKTNVDIEKVMITDEEEIRTTNPVATEQYGSVSTNLQRGNRQAATADVNTQGVLPGMVWQDRDVYLQGPIWAKIPHTDGHFHPSPLMGGFGLKHPPPQILIKNTPVPANPSTTFSAAKFASFITQYSTGQVSVEIEWELQKENSKRWNPEIQYTSNYNKSVNVDFTVDTNGVYSEPRPIGTRYLTRNL

SEQ ID NO: 17 - protein, 736 aa, adeno-associated virus 6
MAADGYLPDWLEDNLSEGIREWWDLKPGAPKPKANQQKQDDGRGLVLPGYKYLGPFNGLDKGEPVNAADAAALEHDKAYDQQLKAGDNPYLRYNHADAEFQERLQEDTSFGGNLGRAVFQAKKRVLEPLGLVEEGAKTAPGKKRPVEQSPQEPDSSSGIGKTGQQPAKKRLNFGQTGDSESVPDPQPLGEPPATPAAVGPTTMASGGGAPMADNNEGADGVGNASGNWHCDSTWLGDRVITTSTRTWALPTYNNHLYKQISSASTGASNDNHYFGYSTPWGYFDFNRFHCHFSPRDWQRLINNNWGFRPKRLNFKLFNIQVKEVTTNDGVTTIANNLTSTVQVFSDSEYQLPYVLGSAHQGCLPPFPADVFMIPQYGYLTLNNGSQAVGRSSFYCLEYFPSQMLRTGNNFTFSYTFEDVPFHSSYAHSQSLDRLMNPLIDQYLYYLNRTQNQSGSAQNKDLLFSRGSPAGMSVQPKNWLPGPCYRQQRVSKTKTDNNNSNFTWTGASKYNLNGRESIINPGTAMASHKDDKDKFFPMSGVMIFGKESAGASNTALDNVMITDEEEIKATNPVATERFGTVAVNLQSSSTDPATGDVHVMGALPGMVWQDRDVYLQGPIWAKIPHTDGHFHPSPLMGGFGLKHPPPQILIKNTPVPANPPAEFSATKFASFITQYSTGQVSVEIEWELQKENSKRWNPEVQYTSNYAKSANVDFTVDNNGLYTEPRPIGTRYLTRPL

SEQ ID NO: 18 - protein, 599 aa, adeno-associated virus 6
TAPGKKRPVEQSPQEPDSSSGIGKTGQQPAKKRLNFGQTGDSESVPDPQPLGEPPATPAAVGPTTMASGGGAPMADNNEGADGVGNASGNWHCDSTWLGDRVITTSTRTWALPTYNNHLYKQISSASTGASNDNHYFGYSTPWGYFDFNRFHCHFSPRDWQRLINNNWGFRPKRLNFKLFNIQVKEVTTNDGVTTIANNLTSTVQVFSDSEYQLPYVLGSAHQGCLPPFPADVFMIPQYGYLTLNNGSQAVGRSSFYCLEYFPSQMLRTGNNFTFSYTFEDVPFHSSYAHSQSLDRLMNPLIDQYLYYLNRTQNQSGSAQNKDLLFSRGSPAGMSVQPKNWLPGPCYRQQRVSKTKTDNNNSNFTWTGASKYNLNGRESIINPGTAMASHKDDKDKFFPMSGVMIFGKESAGASNTALDNVMITDEEEIKATNPVATERFGTVAVNLQSSSTDPATGDVHVMGALPGMVWQDRDVYLQGPIWAKIPHTDGHFHPSPLMGGFGLKHPPPQILIKNTPVPANPPAEFSATKFASFITQYSTGQVSVEIEWELQKENSKRWNPEVQYTSNYAKSANVDFTVDNNGLYTEPRPIGTRYLTRPL

SEQ ID NO: 19 - protein, 534 aa, adeno-associated virus 6
MASGGGAPMADNNEGADGVGNASGNWHCDSTWLGDRVITTSTRTWALPTYNNHLYKQISSASTGASNDNHYFGYSTPWGYFDFNRFHCHFSPRDWQRLINNNWGFRPKRLNFKLFNIQVKEVTTNDGVTTIANNLTSTVQVFSDSEYQLPYVLGSAHQGCLPPFPADVFMIPQYGYLTLNNGSQAVGRSSFYCLEYFPSQMLRTGNNFTFSYTFEDVPFHSSYAHSQSLDRLMNPLIDQYLYYLNRTQNQSGSAQNKDLLFSRGSPAGMSVQPKNWLPGPCYRQQRVSKTKTDNNNSNFTWTGASKYNLNGRESIINPGTAMASHKDDKDKFFPMSGVMIFGKESAGASNTALDNVMITDEEEIKATNPVATERFGTVAVNLQSSSTDPATGDVHVMGALPGMVWQDRDVYLQGPIWAKIPHTDGHFHPSPLMGGFGLKHPPPQILIKNTPVPANPPAEFSATKFASFITQYSTGQVSVEIEWELQKENSKRWNPEVQYTSNYAKSANVDFTVDNNGLYTEPRPIGTRYLTRPL

SEQ ID NO: 20 - protein, 736 aa, adeno-associated virus 9
MAADGYLPDWLEDNLSEGIREWWALKPGAPQPKANQQHQDNARGLVLPGYKYLGPGNGLDKGEPVNAADAAALEHDKAYDQQLKAGDNPYLKYNHADAEFQERLKEDTSFGGNLGRAVFQAKKRLLEPLGLVEEAAKTAPGKKRPVEQSPQEPDSSAGIGKSGAQPAKKRLNFGQTGDTESVPDPQPIGEPPAAPSGVGSLTMASGGGAPVADNNEGADGVGSSSGNWHCDSQWLGDRVITTSTRTWALPTYNNHLYKQISNSTSGGSSNDNAYFGYSTPWGYFDFNRFHCHFSPRDWQRLINNNWGFRPKRLNFKLFNIQVKEVTDNNGVKTIANNLTSTVQVFTDSDYQLPYVLGSAHEGCLPPFPADVFMIPQYGYLTLNDGSQAVGRSSFYCLEYFPSQMLRTGNNFQFSYEFENVPFHSSYAHSQSLDRLMNPLIDQYLYYLSKTINGSGQNQQTLKFSVAGPSNMAVQGRNYIPGPSYRQQRVSTTVTQNNNSEFAWPGASSWALNGRNSLMNPGPAMASHKEGEDRFFPLSGSLIFGKQGTGRDNVDADKVMITNEEEIKTTNPVATESYGQVATNHQSAQAQAQTGWVQNQGILPGMVWQDRDVYLQGPIWAKIPHTDGNFHPSPLMGGFGMKHPPPQILIKNTPVPADPPTAFNKDKLNSFITQYSTGQVSVEIEWELQKENSKRWNPEIQYTSNYYKSNNVEFAVNTEGVYSEPRPIGTRYLTRNL

SEQ ID NO: 21 - protein, 599 aa, adeno-associated virus 9
TAPGKKRPVEQSPQEPDSSAGIGKSGAQPAKKRLNFGQTGDTESVPDPQPIGEPPAAPSGVGSLTMASGGGAPVADNNEGADGVGSSSGNWHCDSQWLGDRVITTSTRTWALPTYNNHLYKQISNSTSGGSSNDNAYFGYSTPWGYFDFNRFHCHFSPRDWQRLINNNWGFRPKRLNFKLFNIQVKEVTDNNGVKTIANNLTSTVQVFTDSDYQLPYVLGSAHEGCLPPFPADVFMIPQYGYLTLNDGSQAVGRSSFYCLEYFPSQMLRTGNNFQFSYEFENVPFHSSYAHSQSLDRLMNPLIDQYLYYLSKTINGSGQNQQTLKFSVAGPSNMAVQGRNYIPGPSYRQQRVSTTVTQNNNSEFAWPGASSWALNGRNSLMNPGPAMASHKEGEDRFFPLSGSLIFGKQGTGRDNVDADKVMITNEEEIKTTNPVATESYGQVATNHQSAQAQAQTGWVQNQGILPGMVWQDRDVYLQGPIWAKIPHTDGNFHPSPLMGGFGMKHPPPQILIKNTPVPADPPTAFNKDKLNSFITQYSTGQVSVEIEWELQKENSKRWNPEIQYTSNYYKSNNVEFAVNTEGVYSEPRPIGTRYLTRNL

SEQ ID NO: 22 - protein, 534 aa, adeno-associated virus 9
MASGGGAPVADNNEGADGVGSSSGNWHCDSQWLGDRVITTSTRTWALPTYNNHLYKQISNSTSGGSSNDNAYFGYSTPWGYFDFNRFHCHFSPRDWQRLINNNWGFRPKRLNFKLFNIQVKEVTDNNGVKTIANNLTSTVQVFTDSDYQLPYVLGSAHEGCLPPFPADVFMIPQYGYLTLNDGSQAVGRSSFYCLEYFPSQMLRTGNNFQFSYEFENVPFHSSYAHSQSLDRLMNPLIDQYLYYLSKTINGSGQNQQTLKFSVAGPSNMAVQGRNYIPGPSYRQQRVSTTVTQNNNSEFAWPGASSWALNGRNSLMNPGPAMASHKEGEDRFFPLSGSLIFGKQGTGRDNVDADKVMITNEEEIKTTNPVATESYGQVATNHQSAQAQAQTGWVQNQGILPGMVWQDRDVYLQGPIWAKIPHTDGNFHPSPLMGGFGMKHPPPQILIKNTPVPADPPTAFNKDKLNSFITQYSTGQVSVEIEWELQKENSKRWNPEIQYTSNYYKSNNVEFAVNTEGVYSEPRPIGTRYLTRNL

SEQ ID NO: 23 - protein, 6 aa, Homo sapiens
GRGDSP

SEQ ID NO: 24 - DNA, 21 bp, synthetic construct
  source 1..21: mol_type = other DNA
catgtacgttgctatccaggc

SEQ ID NO: 25 - DNA, 21 bp, synthetic construct
  source 1..21: mol_type = other DNA
ctccttaatgtcacgcacgat

SEQ ID NO: 26 - DNA, 20 bp, synthetic construct
  source 1..20: mol_type = other DNA
gaccactaccagcagaacac

SEQ ID NO: 27 - DNA, 19 bp, synthetic construct
  source 1..19: mol_type = other DNA
gaactccagcaggaccatg